European Patent Application EP 4 737 475 A1, published May 6, 2026. Title: Protein variants and a method for producing L-isoleucine using the same. Applicant: CJ CheilJedang Corporation. The sequence listing filed with the application follows.

SEQUENCE LISTING (118 sequences)

SEQ ID NO: 1 - protein, 478 aa, synthetic construct
  REGION 1..478: note = protein variant of gene NCgl0337
MELREYATILMKNWVLIVIASILGIAAGAGFSLLATPEYQSRTQLYVSVRSGAGTTSDMVQGANFSRQIVNSYVDVIKTGVVLEPVVDELGLELTANQLSSHISAASPADTALINITASSPSPQQAAEIANAVGESFKNVIQTELEPDSGDGMSPINLTTTQVALEPSSPVSPNVMMNILLGLLVGLAIGVGIAVLRAALDTRIHSLRDIEEVTDKPLLGGIIADSEVEKHPLIIKHKPHSPIAESFRALRTNLQFLNVGGSSSVFVISSANPGEGKSTTSVNLALALAEAGSRVALIEADLRLPRVSKYLGVEGNAGLTDILIGKAEVNDVLQRWGRTQLYYLPAGRIPPNPSELLGSAEMDKVIAELEESFDYVIIDAPPALAVTDAAVIGHGKAGILIAVSAGSTKKPELEATLSTLENADANVVGVVATMLPPKSVAGYGYGNYGYGDTSKINAPKPDNTELTTTDASKANNEQ

SEQ ID NO: 2 - protein, 469 aa, synthetic construct
  REGION 1..469: note = protein variant of gene NCgl0658
MAKRIVIIGGGPAGYEAALAGAKYGADVTVIEDVGVGGSAVTMDCVPSKSFIAGTGIKTDLRRADDMGLNRGLGKAHLEIDALNIRVKDLAKAQSEDILGQLQRSDVRMINGVGRFDDYNTKQTTHYIKVTHSDGSEETVECDLVLVATGATPRILKGAEPDGERILTWRQVYDIEELPTHLIVVGSGVTGAEFVSAFAELGVKVTMVASRDRILPHDDADAADVLETVLAERGVSLEKHARVESVTRTEDGGVCVRTADGREIYGSHALMTVGSIPNTADLGLENIGVELAPSGHIKVDRVSRTNIPGVYAAGDCTDLFPLASVAAMQGRIAMYHALGEGVSPIRLKTVATAVFTRPEIAAVGITHAQVDSGEVSARVIVLPLATNPRAKMRSLRHGFVKLFCRRNSGLIIGGVVVAPTASELILPIAVAVTNRLTVADLADTFAVYPSLSGSITEAARQLVQHDDLG

SEQ ID NO: 3 - protein, 716 aa, synthetic construct
  REGION 1..716: note = protein variant of gene NCgl0674
MGTARGLSQVLKEARQGGKPTSATQKVPRSGYRYDLDGLRGIAIAFVVLFHVFVGKVSGGVDVFLLLSGYFFLGSQLRYADRPDSSINPWWPIWRTLRRLLPALVLVLGVSMVLILAWVPRLQRIEIANQAVASLFYVQNWELASQGAAYGAASAEVSPFQHLWSMAVQGQFYLFAILLSMTIILIRRYRPEYSAVRLATPVLAVLTSVSFFSAILWHFIDQSVNYYSTFTRFWELGLGALLVLHAPRILISAKTKSILAAVGLFMVLSTGFFMDGAETFPGFPALYPILGACLVILGDGKISVFLSRKWMLWLGDIAYPLYLWHWPLLIIFTALFNQEEPSIWLGIAVIMLSLGLAQLTNKYVEKPMQQQGKRPLFRESRSADALQKLRSSRPARMRAYAGIAVVAVGFALTSTPQVLYQRVLDTQMSDLDPEIYPGALSLAGFDAPEVKPKPNPYVLADTVSPAWAKGCMSVFGDDPSELAPDNYDEDYCAFGNPNSPVEVYLVGGSHAEQWMAPLDALGKQHNFKVIPLVRQSCPTFVVELDGIFSDDCIEFNEKVIERLAEVKPDLVVSNSTRPLLEKGRGIDEVPESYITLWDFLEAEDIPFMGLRDNPWFIQPGGEGWMVSQCYEEEQSLVDCSITKDNFYAPVDPAEKELAIRNNMLAVDTSRWFCPDDLCIPVIGNVYVYRDGNHMSDEYAQSLAPFLWSNMRRLLVA

SEQ ID NO: 4 - protein, 264 aa, synthetic construct
  REGION 1..264: note = protein variant of gene NCgl0686
MSTAYFIAHGNDTYRPTEHSSGAWRDDELHLAPVAGLVIHHMERWRREVVGDALVFSRFSLEVLGQIARDDVTLRTEIVRPGRTIELIETVAEINGRVTIRARAWLLKTSDLAHISGDTFEALPSMTELADVKSAFQWSGGFMDSIVFVEDAEKIPGKNRAWITGDVQLVDGEDSEPLAEFSKFLDVANGVAVREDPKTWMFPNVDLTFHLFRQPVGTKVGFDTRAAFGPNGIGLTTSVIHDAEGPVGTLNQSLTVRPIAELNK

SEQ ID NO: 5 - protein, 1532 aa, synthetic construct
  REGION 1..1532: note = protein variant of gene NCgl0706
MSAFDSILNVEEWISDHYLTNDDAKGASFSKRVRERIKEWKTTEDATQQSGPLTRFSSNRLQLQHALSELDDATTAASLVASALGYGVPSARHAQRGSDTISYSSWVGNAGSVEFLAATPAESFEENFRSLPLEPVAVNDKPQDITAAKLVGQIFLSDTPPAFVVITAGKWVVLAERETWPLGRHLAIDISLVVERNDTKAQGEMQQTVVALARENTERAADGTTWWEETIEQSREHAVKVSGELRSAVRESIEILGNDVLTRYEAKELSTAEIDGGELAKQSLRYLYRILFLLFAEASPELEILPTGTPEYDEGYGLARLRELILNPPVTQHARTGTHLYDSLQLLFTLVDKGHHPTDAKAVAFDAEAGEEGLHFRNLSADLFLPAATELIDRVGLSNEALNKVLENLLLSRVQSGKDRGFISYATLGVTELGQVYEGLMSYTGFIAQEDLFEVAPHGKADKGSWMLPVSKADEVPADSFIEVDQEAPGGGVIKVRKRHPRGSFVFRQSSRDRERSASFYTPQVLTSFTVTQAIEELQASKRITTANDVLSLTICEPAMGSGAFAVEAVRQLAELYLELRQEELEQQIPAEDRAKELQKVKAHIALHQVYGVDLNSTAVELAEISLWLDTMNAEMDAPWYGLHLRNGNSLVGATRSLYAPSLLNKKAWLTATPTRYRLDDIAQAIDENKAEPLFNHGIHHFLLPSTGWGATADAKDLKDLMATEIKELKSWRTSIRASLSKTQIKQLNNLALRVETLWRFVLMRIRIAESQISRSTTLWGQEPAEVSEVVTREQIEQDLFGNIDGAYNRLRLVMDAWCALWFWPLDAVATAEHPERPALPDLDEWLATLTEILGIDLPLKSKNENQIVLGPDTNWLAINDAEATDLGFSGALSFERVSANHPWINVARQVAKQQSFFHWDLDFAHVFAKGGFDLQVGNPPWVRPDVNFEDLLAEHDPWWAVMSKPTQASKKERQKNFHNNPKSLEHVVSGAGETVATSAILGSVTLYPHLKDQRPDLYRGFMEKTWSNASPAGAISLIHPESHFTEKKAAPLRRGAYERLRRHWQFINELILFDVHDLVKYGVHVYGAPQESINFLSAASLYHPQTVLDSFDHDGSGNLPGLKDDNGNWDRRPHKDRIQLVNADTLTVWKSILEDEQTPYLDTRMVYTVNTEAAAVLEKLASAPRIKELGLQFSSGWNETTDKKKGYFDVGWGYPASWSDAILQGPHLGVATPMIKQPNPTMKHNQDWSEIDFEAIPANFIPATAYQPDRQTKPTYDADYGTWTFGDKQVPVADTFRIAWREMAATTGFRTVYPSVIPPGANHVHTVNSAASRSNLKTILVGAQLGAILSDYFARSSGSSHIFNDIVRKIPLPNFTSLEKQFARTYLRLNCLTSAYAPLWEEITGEPWDVQVPLRNAEQRRAAQNDIDAMVALSLGISADELCMIYRTQFPVMRRYDQEDHFDANGRKVPKEIIKLQQKLKDGQELSVEKRTWVHPQSEVSYTFEYPFRVLDREADLRAAYAKFENQLKEP

SEQ ID NO: 6 - protein, 483 aa, synthetic construct
  REGION 1..483: note = protein variant of gene NCgl0885
MRKGISRVLSVAVASSIGFGSVLSGTGIAAAQDSAFDYGMDPSMNYNPIDDIKDRPQGLSNLPYFGSKLTSWGSSDATASSGVVTSALPQYTDPRYPLGKDDLPKATIDMEPEVLARLERFVGVDGDRIRQINAYSPSMGRTIPLVWVVPEDNTVPGPTVYALGGGDGGQGGQNWVTRTDLDELTSENNINLIMPMLGSFSFYADWAGESESMGGAQQWETFLMHELPEPLEAAIGADGQRSIVGMSMSGGSVLNFATHDPNFYSSVGSFSGCAETNSWMGRRGIAATAYNGNVVPEQIFGEVDSDYSRYNDPLLNAAKLEEQDNLYIFAGSGVFSELDVIGDNAPIDEDAFKNRVLVGFEIEAMSNTCTHNLKAATDQMGIDNINYDFRPTGTHAWDYWNEALHRFFPLMMQGFGLDGGPIPIYNPNGVTSSESSSELSSDVSLGTVIGSVAGSSGSSAGSSVREFIAGSSGSSQSAGSFYE

SEQ ID NO: 7 - protein, 520 aa, synthetic construct
  REGION 1..520: note = protein variant of gene NCgl1142
MTTTTSSGKSSEKINPLFKLGSFLRKGTVGSEGQQIFLQGGRQADVFYRNRWAFDKVVRSTHGVNCTGSCSWKVYVKDGVITWESQAVDYPTTGADMPDYEPRGCPRGASFSWYTYSPTRIRYPYIRGVLVDMYREAKERLGDPVLAWRDIVETPEKRKAYVSQRGKGGLIRVQYEEAMEIAAAAHVYTIRQYGPDRIHGFTVIPAMSQVSYGAGTRFLQMIGGVALSFYDWYADLPPASPQTFGDQTDVPESGDWYNSSYLMMWGSNIPVTRTPDSHFMVEARYKGTKVVVVSPDFADSTKFADEWARIHPGTDGALAFAMGHVILKEFHVDKKTPYFMDYMRKYTDSPFLVELDEHGDGTYTPGKFLTADRAADISPALAATPNATHRLLVLQKDGSVVDPGGTVADRWGEEGMGKWNLRLDGVDPVMTIADVQTDTETAEVLFPRFDLPATATQEGPIGAGTISRGVPTITLNGRKYTTVFDVLLAHYGVNREELNLPGEWPKDFQDPVMGTPAWQE

SEQ ID NO: 8 - protein, 483 aa, synthetic construct
  REGION 1..483: note = protein variant of gene NCgl1165
MTTALEEQNAQQAATAGRVVRVIGAVVDVEFPRGELPALYNALTVEVTLESVKKTVVLEVAQHLGDNLIRTIAMAPTDGLVRGAAVTDTARPISVPVGDVVKGHVFNALGDCLDDVSLNNNPEIERWGIHREPPSFDQLEGKTEILETGIKVIDLLTPYVKGGKIGLFGGAGVGKTVLIQEMITRIAREFSGTSVFAGVGERTREGTDLFLEMEEMGVLQDTALVFGQMDEPPGVRMRVALSGLTMAEYFRDVQNQDVLLFIDNIFRFTQAGSEVSTLLGRMPSAVGYQPTLADEMGVLQERITSTKGRSITSLQAVYVPADDYTDPAPATTFAHLDATTELDRSIASKGIYPAVNPLTSTSRILEPAIVGERHYEVSQRVIGILQKNKELQDIIAILGMDELSEEDKITVARARRIERFLGQNFFVAEKFTGLPGSYVPLTDTVDAFERICNGDFDHYPEQAFNGLGGLDDVEAAYKKLTGK

SEQ ID NO: 9 - protein, 587 aa, synthetic construct
  REGION 1..587: note = protein variant of gene NCgl1253
MTPTQNEIHPKHSYSPIRKDGLEVPETEIRLDDSPSGPNEPFRIYRTRGPETNPKQGLPRLRESWITARGDVATYQGRERLLIDDGRSAMRRGQASAEWKGQKPAPLKALPGKRVTQMAYARAGVITREMEFVALREHVDAEFVRSEVARGRAIIPNNVNHPESEPMIIGRKFLTKINANIGNSAVTSSIEEEVSKLQWATRWGADTVMDLSTGDDIHTTREWIIRNSPVPIGTVPIYQALEKVNGVAADLNWEVFRDTIIEQCEQGVDYMTIHAGVLLAYIPLTTRRVTGIVSRGGSIMAGWCPAHHRESFLYEHFDELCEIFAQYDVAFSLGDGLRPGSLADANDAAQFAELKTIGELTQRAWEYDVQVMVEGPGHVPLNMIQENNELEQKWAADAPFYTLGPLVTDIAPGYDHITSAIGAAHIAMGGTAMLCYVTPKEHLGLPNRDDVKTGVITYKLAAHAADVAKGHPGARAWDDAMSKARFEFRWNDQFALSLDPDTAIAYHDETLPAEPAKTAHFCSMCGPKFCSMRISQDIRDMFGDQIAELGMPGVGDSSSAVASSGAREGMAEKSREFIAGGAEVYRR

SEQ ID NO: 10 - protein, 720 aa, synthetic construct
  REGION 1..720: note = protein variant of gene NCgl1315
MLARCFAAGRNVSTLWRILECMAFAAEHPVLSHSEHRPVGEIERSDDKFVVVSEFEPAGDQPAAIKELDERLDRGERDVVLMGATGTGKSATAAWLIEKQQRPALVMAPNKTLAAQLANELRQLLPNNAVEYFVSYYDYYQPEAYIAQTDTYIEKDSSINEDVERLRHSATSSLLSRRDVVVVSSVSCIYGLGTPQSYLDRSVVLNVGEEIDRDRFLRLLVDIQYERNDVGFTRGAFRVKGDTVDIIPAYGELAVRIEFFGDEIDALYYIHPLTGDTIRQVNEIRIFPATHYVAGPERMEKAVADIKAELEVRLADLENRGKLLEAQRLRMRTEYDLEMIEQVGFCSGIENYSRHIDGRGEGTAPATLIDYFPEDFLTIIDESHVTVPQIGGMFEGDMSRKRNLVEFGFRLPSAMDNRPLTWEEFDERRGQTVFMSATPGKFEIAAADGEFVEQVIRPTGLVDPKVTVKPTKGQIDDLIHEIRQRTDKDERVLVTTLTKKMAEDLTDYLLENGIRVRYLHSDIDTLQRVELLRQLRLGEYDVLVGINLLREGLDLPEVSLVAILDADKEGFLRSTTSLIQTIGRAARNVSGEVIMYADKITDSMQYAIEETDRRREKQVAYNKEHGIDPQPLRKKIADILDQVYDNSADGAGPSASGDAAVVAKPDVSSMPAKEVQKLIDDLSAQMAAAARELKFELAGRLRDEIFELKKELRGIKDAGI

SEQ ID NO: 11 - protein, 323 aa, synthetic construct
  REGION 1..323: note = protein variant of gene NCgl1511
MGDLKMQRSGGEPLDTIKAYIALTKPRVIELLLVATIPTMLQAERGENNIVLILLTVFGGWMGAAAANTFNMVADSDIDQRMGRTRARPLVRHTVSNRDASIFAWVLTVASFLWLWLLCDSMLAGIFVLITIFFYIFVYTKWLKRRTHMNIVWGGAAGCMPVLVGWAVIVDQFEPGVPQQWWQAIVLFMVIFFWTPPHTWALAMKYREDYKAAGVPMLPVVRTPVQVTAQIVWYSVATVLTTFLLIPATGWIYAAIAVISGVTFLFMAIKLHLGIKNGGKVKPLKLFILSNNYLAVLFVALSVDAVLGLETIGEMLGWTTTFF

SEQ ID NO: 12 - protein, 185 aa, synthetic construct
  REGION 1..185: note = protein variant of gene NCgl1588
MKLFSRTSLVALGTAAAITLSGVTAPAFADEDSNAAVSALKTAEDNTPEAPGASTPLKLEQPGTITGVPGKAITPVTVKVIAGEAESFTSDNLPSGLLIDNTGKITGTPKKEFTGSAKIIAKNEAGVEAEVYVNFDFNEEPSSEEPSSGSSDTDNIENWIKIITAVIGALTTILTFSTKLDSFLK

SEQ ID NO: 13 - protein, 528 aa, synthetic construct
  REGION 1..528: note = protein variant of gene NCgl1815
MRSDVIELPEGVSKDEADQVEVAEARLNEGARLMAATGCEAMWPTGFSVCGRILDAYRQVGGQLSWLGPPKSNELTNPDGVGKRSEFFGGAIYWHPDTGAYAVTLDGLRQWGTLNWESGPLGYPTSGPMDTNYPLTQRQTFQGGDNYYNPLTGGAVWGDIKQRYEELGGSNHAIGIPITNELPSGTEYFYNNFSNGTISWRNDRQTRFMYLATQRVWDALGRETGRLGFPEADETPEVSGLFHVVNFAERGVIAWNGILGARELYGDVYSLWLQYQNTDTPLGWPIPSLTSLNESLEQEFTRGVVLGSGDALTWIPDDEERSLEDFLPIGSSGSSSSSQEMTLFSQRAQYVDCKNLPDLDEQRKTENNIEKNGGPIKKEYSSRGFPTEFRFVVRKGHYDRYRNEGWGYLKNYCKHNFANHAMAEAVVDKAVIDYGSSPGTSYYKFEKTVYFLDCRTYTFNKNSGCKEMHAPQWVTIIYNPHTFTGANSNRPKGVISAWCNSTPPGGIEHEPEISQCPDHVNLYNKLRI

SEQ ID NO: 14 - protein, 264 aa, synthetic construct
  REGION 1..264: note = protein variant of gene NCgl1859
MVSQTERQHAIASLLAPTGAVSVGDLAEHFHVTTETVRRDLRIMESLGLLQRVHGGAISPEPMGTSPPRLKPALVKGMPPEPRVLELAETAVSLITPLARSIFLDSGLACTAIATVLGDPPEDARWTVVTSSPGAVIALSATDATSTVVLHGQVHGNCSSIIGSTAVDMISQLRADIAFVEVDAIQSDTSLCTFFPETIPIKQAMIKNAAFTVAVLSPRSPQDQELQLLKHPFSTLADFDALVTDDHTLDFPVLPDHNFQVVTP

SEQ ID NO: 15 - protein, 526 aa, synthetic construct
  REGION 1..526: note = protein variant of gene NCgl1874
MTQQLNHAKVNQHPGQATLPETAEGQVRTYEVKTYGCQMNVHDSERLSGLLEEAGYVAAPEDTTPDLVVFNTCAVRENADMRLYGTLGNLRSVKEKNPGMQIAVGGCLAQKDKDTVVKKAPWVDVVFGTHNIGSLPTLLQRAEHNAQAEVEIVDSLEQFPSVLPAKRESAYAGWVSVSVGCNNTCTFCIVPSLRGKEQDRRPGDILAEVQALVDQGVTEVTLLGQNVNAYGVNFVDPELERDRSAFSKLLRACGEIEGLERVRFTSPHPAEFTSDVIDAMAETPNICPQLHMPLQSGSDKVLKEMRRSYRSKKFLSILDEVRAKIPHASITTDIIVGFPGETEEDFQATLDVVKKARFTSAYTFQYSPRPGTPAAEYENQLPKEVVQERYERLMVVQEQVCEEENQKLIGTTVELLVQAGGGRKNDATKRMSGRARDGRLVHFAPEGDIDGEIRPGDFVTVTVTEAKPFFLIADSGVQTHRRTKAGDNSAVGQVPTTAPIGVGLGLPQIGAPKVAPATESACCSIN

SEQ ID NO: 16 - protein, 324 aa, synthetic construct
  REGION 1..324: note = protein variant of gene NCgl2245
MSKTEEGRSAAIIIYAFPTFILLGAIIAFIFPEPFIPLTNYINIFLTIIMFTMGLTLTVPDFQMVLKRPLPILIGVVAQFVIMPFLAIVVAKMFNLNPALAVGLLMLGSVPGGTSSNVIAFLARGDVALSVTMTSVSTIVSPIMTPFLMLMLAGTETAVDGGGMAWTLVQTVLLPVIIGLVLRVFLNKWIDKILPILPYLSILGIGGVVFGAVAANAERLVSVGLIVFVAVIVHNVLGYVVGYLTGRVFKFPEAANRTMAIEIGTQSSGLASGMAGRFFTPEAALPGAVAALVHNITGAVYVGLVRNRPLTKASRKKESVAVSS

SEQ ID NO: 17 - protein, 293 aa, synthetic construct
  REGION 1..293: note = protein variant of gene NCgl2580
MSFTAFQTALLVWFRANARDLAWRDPNTSAWGILLSEVMSQQTPVARVEPIWREWMEKWPTPEDFANASTDEILRSWGKLGYPRRALRLKECAEVIVEKHAGEVPDTVEALLALPGIGDYTARAVAAFHFGQRVPVVDTNVRRVYQRAVAGRYLAGPAKKQELIDVSLLLPNTHAPEFSAAIMELGALICTATSPKCDTCPLLDQCQWQKLGCPSPSEEELASAKKRVQKFVGTDRQVRGLIMDVLRNATAPVPLSAIDVVWPDDAQRSRALFSLIEDGLAEQDEAGYFHLPR

SEQ ID NO: 18 - protein, 893 aa, synthetic construct
  REGION 1..893: note = protein variant of gene NCgl2629
MVNTLNSKTVNVPRFARGVVAAATALFFGALVSLAPSALAQEPPAVEAGASGSLSNLGACIADKGTLDVIIMIDETESLIHEARDGVVNANEPGADAQHHRVPAAQSFVDELLAKQSDGDLNTRIRVAGFGQTYKSGATDPDNYGAWTQLDASTVGGVQDEISRFADRTQEQYTNYASAIEGAYQDFTRSGSEDACRMLVTFTDGALTAQEGADVAEAALCAPGGVTDRLRSAGITHIGIGLSAPTNPSDFSLLRGTTAGGGTCGVEPANGAFFPADNVGGLFAAFREALAIGGETIGETRAGDPFSFTLDNSVNSVRFTAIAKDDLGPNAHLVLTAPNGETVELKDSGSSVANSTDVSWEAESSPVKMADGSLNLQQGGDWKGVWQIQFQGIDPAAVDGRVFNSVEIQPDLQLVFSGGDSTSGALNLRDDQQLNMQLVGRDGQPRILEGSALVDLGFTRADTGEFAPLAQGIDISGGELSFPLDTISQLPAIGTVEARTTITTAGVDDLPGTTLSPILNTTRITITQRDMPQLPASVRFTADEDVVTVDIPITGPGKVWIAPGTQLSGVLPDGVDGIAASSTFDSPDNALVLGLDEQGTIPVELTVSDLRDGLVNGSIPLQISNAEGANETSVDLPTEGTLSVPINASTFALAFILALVLSLLIPLLILYIVRFLSAKVPSSAMSGVRIPVEFSGEALRYAGSTMPDLASQTTATKQVVVHGDTFNVEGHKLKVQRFQLNPIASPAVIVQTDPSISFDGKQKGTQAKLPLAVQGSWFLTASGADPSKMELIALTNLPLEQGQIDRMIAGITSKAPDRARELQKLLDDAATSQPAKVPPRAPAAQGHVEKQAPSFGTGSGGVFGSSNGGGFGSGSGSNDTNGGFGSSGGFGAR

SEQ ID NO: 19 - protein, 240 aa, synthetic construct
  REGION 1..240: note = protein variant of gene NCgl2863
MADRTPTTATPPGWVLVVDDEQPLAQMVASYLIRAGFDTRQAHTGTQAVDEARRFSPDVVVLDLGLPELDGLEVCRRIRTFSDCYILMLTARGSEDDKISGLTLGADDYITKPFSIRELVTRVHAVLRRPRTSTTPPQVTTPLIVGDLILDPVAHQVWVGETTVELTRTEFELLVALALRPGQVLTRHDLITEVWDTTWVGDERIVDVHIGNLRRKLGTDTRGRGFIDTVRGVGYRVGQP

SEQ ID NO: 20 - DNA, 1437 bp, synthetic construct
  misc_feature 1..1437: note = nucleotide variant of gene NCgl0337
  source 1..1437: mol_type = other DNA
atggaattaagggaatacgcgacaatcctgatgaagaattgggtgttgatcgttatcgcatccattcttggaattgcagcgggcgctggtttttcccttctagctacaccggagtatcagtcacgtactcagttgtatgtatcggtgcggtcgggggctgggacaacctctgacatggttcagggtgctaacttttcgcgtcagattgtgaatagttatgttgatgtcattaagacgggtgttgttctagagccggttgttgatgagcttggtctggagttgacggctaaccagttgagttctcatatcagtgcggcttctcctgctgatactgcgttgatcaacatcactgcttctagtccttctcctcagcaggcggctgagatcgccaatgcagtgggggagagtttcaagaatgtgattcagactgaattggaaccagactccggcgatggcatgagcccgattaacctgactactactcaggtggctctggaaccatcttctccggtcagtcctaatgtgatgatgaatatcctcctcggcctacttgtaggtcttgcaataggtgttggtattgcagtgcttcgcgcggctttggatactcgtattcattccttgcgcgatattgaagaggttactgataagccacttttgggcggaatcattgcggattctgaagttgagaagcacccgttgatcattaagcacaagccgcatagtcctattgcggagtcctttcgtgcgttacgtactaacctgcagttccttaacgtcggcggctcatcttcagtatttgttatctcctctgctaatcctggtgagggtaagtcaaccacttctgtaaacctagctttggcgcttgcagaggccggctcccgtgtagcgctgatcgaagctgatcttcgcttgccacgagtgagcaagtacctcggagttgagggcaacgcaggtctgactgacattctcattggcaaggccgaggttaatgatgtgttgcagcgttggggtaggactcagttgtactatctcccggcagggcgcattccgccgaacccgagtgagttgcttggttcagctgagatggacaaggtcattgcggagcttgaggaaagctttgattatgtgatcatcgatgcccctccggcgttggcggttaccgatgctgcagttattggtcatggcaaggctggcatcctgattgcggtctccgcaggttctacaaagaagcctgagttggaagctacgctgtccacgcttgagaatgcggatgccaatgttgttggcgttgtcgctacgatgctcccgcctaagtctgtggctggttatggctacggaaattacggctacggcgacacctccaaaatcaatgcccctaagcccgacaacaccgaactaaccaccaccgatgcttccaaggccaacaatgagcaatag

SEQ ID NO: 21 - DNA, 1410 bp, synthetic construct
  misc_feature 1..1410: note = nucleotide variant of gene NCgl0658
  source 1..1410: mol_type = other DNA
atggcaaagaggatcgtaattatcggcggtggacctgcaggctatgaagccgcactcgcaggcgctaaatacggtgcagacgttaccgttattgaagatgtcggagttggcggatccgcagtcaccatggactgtgtaccttcaaagtccttcatcgctggtaccggtatcaaaaccgacctccgacgtgctgatgacatgggacttaaccgtgggcttggaaaagcacacctagaaatcgatgcactgaacatccgtgtgaaggaccttgcgaaagcacagtccgaagatatcttgggccagctgcagcgctcagatgtccgcatgattaacggtgtgggccgctttgatgattacaacaccaagcaaaccacccactacattaaagtcacccacagcgatggctccgaagaaaccgttgagtgcgatctggtgctggttgcaactggtgcaaccccccgcattcttaaaggtgcagagccagacggcgagcgcatcttgacctggcgtcaggtctacgacattgaagaactccccacccaccttatcgtggttggttccggtgtgaccggtgcggaatttgtctctgcgtttgctgaactcggcgtcaaagtcaccatggtggcatcccgtgaccgcattttgcctcacgatgacgcagatgccgcagacgtgctggaaaccgttctggctgagcgcggagtatccctggaaaagcatgcccgcgtggagtctgtcacccgcaccgaagacggtggcgtgtgtgttcgcactgctgacggacgagaaatctacggttctcacgcgttgatgactgttggttccattccaaacacggcagatcttggcctggagaacatcggtgttgagctggcaccatccggccatatcaaggttgaccgcgtctcccgcaccaacatccccggtgtgtacgcagcaggtgactgtactgacctattcccactggcgtccgttgcagcgatgcagggccgtatcgccatgtatcacgcactcggtgaaggcgtgagccccatccgtttgaagactgttgccaccgcagtgtttacccgcccagagatcgcagcagtaggtatcacccatgcacaagttgattccggcgaagtgtctgctcgcgtgattgtgcttcctttggctactaacccacgcgccaagatgcgttccctgcgccacggttttgtgaagctgttctgccgccgtaactctggcctgatcatcggtggtgtcgtggtggcaccgaccgcgtctgagctgatcctaccgatcgctgtggcagtgaccaaccgtctgacagttgctgatctggctgataccttcgcggtgtacccatcattgtcaggttcgattactgaagcagcacgtcagctggttcaacatgatgatctaggctaa

SEQ ID NO: 22 - DNA, 2151 bp, synthetic construct
  misc_feature 1..2151: note = nucleotide variant of gene NCgl0674
  source 1..2151: mol_type = other DNA
gtgggaacggcgagagggctttctcaagttctgaaagaagccagacaaggtggaaaacccacttcagccacccagaaagttccacgctccggctacagatatgacctcgatgggctccgcggcatcgcgatcgccttcgtagttttgttccatgttttcgtcggaaaagtctccggcggtgtggatgtcttcctgctgctgtctggctatttcttcttagggtcgcaattgcgttatgcagatcgtccagattcttccatcaacccctggtggccgatttggcgcacgctacgcagattacttcctgcgttagtgctggtgttgggcgtttccatggtcctcatcttggcgtgggtgcccagactgcaacgaatagaaatagccaaccaagcagtagccagcctcttctatgtccaaaactgggagctcgcatcccaaggtgctgcctacggagcagcctctgcagaagtcagtcctttccagcacttgtggtccatggctgtgcaagggcagttctacctctttgccatcttgttgagcatgacgatcatcctgattcgtcgataccgccccgaatactccgcagtgcgactagcgactcctgtgctggcagtgctcacatccgtatcatttttcagtgcaatcctgtggcatttcattgatcaatcagtcaactactattccaccttcaccaggttctgggagctcggccttggtgcactattggtgctgcatgcgcctcgaattttgatttctgcgaagactaaatcaatactcgcagccgtcggtttgtttatggtgctatccactggattcttcatggatggcgcagagactttccctggattccccgcgctgtatcccatcttgggtgcttgcttagtcatccttggcgacggtaaaatctcggtctttctctcccgaaaatggatgctttggctcggcgatatcgcctacccgctctacttgtggcactggcctctgctgatcattttcaccgctttgttcaaccaagaagagccatccatctggctgggtatcgccgtgattatgctgtcccttggcttggcgcagctgactaacaaatacgtagaaaaaccaatgcaacagcagggaaagcgcccactatttagggaatcccgcagtgctgatgctttgcaaaagctgcgttcctccaggcctgcccgaatgcgtgcgtatgcgggtatcgcagtagtcgcagtcggtttcgccctgacatctactccgcaggtgctctaccaacgagtcctcgatacccaaatgagtgatctcgatccggagatctaccccggtgcactctccctggcgggcttcgatgcccccgaagtaaaacccaaaccaaacccctacgtgctggccgataccgtctcacccgcctgggcaaaaggctgcatgtccgtcttcggcgacgatccatctgaactagcaccagacaactacgacgaagattactgcgctttcggcaaccccaactcacccgtcgaggtctacctcgtcggcggatcccacgccgaacaatggatggcaccactcgacgccctaggcaagcaacacaacttcaaagtgatccccctcgtccgccaatcctgccccaccttcgtggtggaactcgacggaattttcagcgacgactgcatcgaattcaacgaaaaagtgatcgaacgcctcgcagaagtaaaacccgacctcgtggtctccaactccaccagaccgctccttgaaaaaggccgcggcatcgacgaagtgccagaatcatacatcacgctgtgggacttcctcgaagccgaagacatcccattcatgggactccgcgacaacccgtggttcatccagccaggaggcgaaggatggatggtgtcccaatgctacgaagaagaacaatccttggtggactgctcgatcaccaaagacaacttctacgcaccagtagaccccgctgaaaaagaactagccatcagaaacaatatgctcgcagtggatacttcacgatggttctgcccagacgacctgtgtatcccagtgatcggcaatgtgtatgtataccgcgacggcaaccacatgtccgatgaatacgcacaatctttggctccattcctgtggagcaatatgcgcaggcttctggtcgcttag

SEQ ID NO: 23 - DNA, 795 bp, synthetic construct
  misc_feature 1..795: note = nucleotide variant of gene NCgl0686
  source 1..795: mol_type = other DNA
atgtcaactgcatattttattgcgcacggaaacgatacgtaccgcccaacggagcattccagcggtgcgtggcgcgatgatgaactccaccttgcaccggttgccggtttggtgattcaccatatggaacgttggcgcagggaagtggttggcgatgctttggtgttcagccgttttagtttggaggtcttgggccagatcgctcgggatgatgtcaccttgagaacagagatcgttcgtcccgggcgcaccattgaacttattgaaaccgtggctgaaatcaacggcagagtgacgattcgtgcacgcgcctggttgctgaagacctctgatcttgcccatatttctggcgatacttttgaagcgttgccgtcaatgactgaactggcagatgttaagtcagcgttccagtggtctggtggatttatggacagcattgtgtttgttgaggacgctgagaaaattccgggcaaaaaccgcgcgtggattaccggcgatgtgcagttggttgacggcgaagattctgagcctttggcagagttttccaaattcttggatgtggccaatggcgtggcggttcgggaagatccaaagacttggatgttcccgaacgtggatcttactttccatctgttccgccagccggtgggcaccaaggtgggttttgatacccgcgcggcgtttggacccaacggcatcggtttgaccacgtcggtgattcacgatgccgaaggtcctgtgggcacgcttaatcaatcattgacagtgcgcccaattgctgagttaaacaagtga

SEQ ID NO: 24 - DNA, 4599 bp, synthetic construct
  misc_feature 1..4599: note = nucleotide variant of gene NCgl0706
  source 1..4599: mol_type = other DNA
atgagtgcatttgattcgatcctaaatgttgaagagtggatcagtgaccactacctcaccaatgacgatgccaaaggtgcctcattttccaagcgggtgcgcgagcgcattaaagaatggaaaaccaccgaggacgcaacccagcagagtggccctttaactcgtttttccagcaaccgcctgcagttgcagcatgctctttctgagcttgacgacgccaccaccgccgccagtttagtggcctctgcactggggtatggtgtccccagcgcgcgccacgcgcagcgcggctccgacacaatatcctattcctcttgggtgggaaatgccggcagtgtggaatttcttgcagcgactcccgctgaaagctttgaagagaacttccgatcccttccccttgagccagtagcggtcaatgacaagccccaggatatcaccgcagccaaattggtgggccagattttccttagtgatactccccctgcttttgttgttatcaccgctggtaaatgggtggttttagccgagcgtgaaacctggcctctaggccgccacctagctattgatatttccctggtggtggaacgtaatgacaccaaagcccagggtgagatgcagcagacggtcgtagcactagcccgcgaaaataccgagcgtgccgccgatggcaccacctggtgggaagaaaccattgagcaatcccgcgaacatgctgtcaaggtttctggcgagctacgcagtgcggtgcgtgaatccattgaaatcctgggcaatgacgtgctcacacgctatgaagctaaagagctctccaccgctgagatcgacggtggcgagctagctaagcaatctttgcgctatctctaccgcattttgttcctgctttttgccgaggcttcaccagagcttgaaatcctgccaaccggcaccccggaatatgacgagggttatggcttggcacgcctgcgcgagcttattcttaatcccccagttacccagcatgctcgcacgggcacccacctttatgattccctgcagctgctgttcactctggtggataaaggccaccacccaacagatgctaaggctgtagcttttgatgccgaggctggagaagaaggcctgcacttccgcaacctttcagcggatctcttcctccctgcagccacagaacttattgatcgagttggtctttccaatgaagccctaaacaaggtcttggaaaacctcctgctctcccgggtgcaatccggtaaagaccgcggctttatctcctatgccaccttgggtgttaccgagcttggccaagtttatgagggtctgatgtcctataccggctttatcgcccaggaagatctttttgaggttgcaccacatggcaaagccgataaaggttcctggatgctcccggtctcaaaggctgatgaagtccctgccgatagctttatcgaagttgatcaagaagcccctggtggcggcgtaatcaaggtgcgtaaacgccacccgcgcggatcatttgtgttccgtcagtcctctcgtgaccgcgaacgctcagcgtccttctacaccccacaagtactcaccagctttactgtcacccaggctattgaagaactccaggcatcaaagcgcatcaccacagccaatgatgttctcagcctcaccatctgtgaacctgccatgggttccggcgccttcgctgtggaagcagtacgccaattagcagagctttatttggaattgcgccaagaagaactagagcagcagattccagcggaagaccgtgccaaggaactccaaaaggtcaaagcgcacattgcgctgcaccaggtttatggtgtggaccttaacagcactgctgtggagttggcggaaatctcgctgtggctagacaccatgaatgcagaaatggacgcaccttggtatggcctgcacctgcgtaatggtaactccctcgttggtgccacccgttcgctgtatgcacctagtctgcttaataaaaaagcctggttaactgctactccaacccgctatcggcttgatgatatcgcgcaggctattgatgaaaacaaagcagaacccctcttcaaccacggcatccaccacttcctcttgccctctactggctggggagccactgcagatgccaaagatcttaaagatcttatggctactgaaatcaaggagcttaaatcttggcgtacttccatccgtgcgtctttgagtaaaactcagattaagcagctcaataaccttgccctacgcgtggaaacactatggcgatttgtgctgatgcgtattcgcattgcagaatcccagatctcacgtagcactactctctggggtcaagagccagctgaggtttcggaggttgtcacacgtgagcaaattgaacaagacctctttggcaatattgatggtgcatataaccgtctacgcttggtgatggatgcttggtgtgcgctgtggttctggcctttggatgctgttgctaccgctgagcatccggagcgtccagcccttccagatcttgatgagtggctagccaccctgacggagattctgggtattgatctccctctgaagtccaaaaacgaaaatcagattgtcttaggtccagataccaattggctagccattaatgatgccgaggctactgatcttggtttttctggggcattgagctttgagcgtgttagcgcgaatcacccgtggatcaatgttgcccgccaagtggctaaacaacagagcttcttccactgggatctagacttcgcccacgtttttgccaagggtggatttgatctgcaggttggtaatccaccatgggtgcgaccagatgtgaactttgaggatctgcttgctgaacatgatccgtggtgggctgtaatgagtaaaccaacccaggcatccaaaaaagaacgccagaagaattttcacaacaatcctaagagcctcgaacatgtggtcagtggtgcaggtgaaaccgtggctacttctgcgatcctcggttcggttactctctatccgcatcttaaagatcaacgcccggacctctaccggggctttatggaaaagacttggtctaatgcctccccggcaggtgcgatctcactgatccaccccgaatcccacttcactgagaaaaaagctgccccgctacgtcggggagcatatgagcgtctgcgccgccactggcagttcattaatgagttgattctttttgacgtccacgacttggttaaatatggcgtacatgtctatggcgctccgcaggaatctattaactttttaagtgctgcgtcgctttatcacccacaaacagtgcttgattcatttgatcatgacggttcaggtaatctccctggtcttaaagacgacaatggcaactgggaccgtcgcccacacaaggaccgtatccaactggtcaatgccgatactttgacggtgtggaagtccatcctggaggatgaacaaacgccatacttggatacccgcatggtttataccgtcaacacggaagcagcagcagtgttggaaaagttggcttctgcacctcgtatcaaagaactcgggctgcagttctccagtggctggaatgaaaccaccgataagaaaaagggatactttgacgttggttggggctacccagcttcctggtctgatgccattttgcaggggccgcacctgggtgttgctacaccaatgatcaagcagcccaatccgacaatgaagcataatcaagattggtctgaaattgatttcgaggccattcctgcaaacttcatacctgcaacggcgtaccagcccgatcgccaaacaaagcccacttatgatgctgactacggcacctggactttcggggacaagcaggtaccagttgcagacactttccgaattgcatggagggagatggctgccaccacgggatttaggactgtctacccatcagtaattccaccgggagccaaccatgtgcacacagttaatagcgctgcatcacgttcaaacttaaaaaccattctcgttggagcacagcttggtgcaattctaagtgactattttgctcggtcctcgggttcaagccacatatttaacgacattgttcgcaagattccacttccaaatttcacatccttggaaaagcagttcgcccgcacatacctccgcctcaactgcctgacctcagcttatgccccattgtgggaagagatcaccggtgagccgtgggatgttcaggtgcctttgcgcaatgccgagcaacgtcgagcagcgcaaaacgatattgatgccatggtggcattgtctttgggtattagtgctgatgagctgtgcatgatttatcgcactcaattcccagtgatgcgtagatatgatcaagaagatcattttgatgccaatggccgtaaagttcctaaagagatcatcaagctgcagcagaaacttaaagatggccaagagctcagcgtggaaaagcgcacctgggtgcatccccaatcagaagtgtcctatacctttgaatatcctttccgggtgttggatcgtgaagctgatctgcgtgctgcatatgcaaaatttgaaaaccagctaaaggagccatag

SEQ ID NO: 25 - DNA, 1452 bp, synthetic construct
  misc_feature 1..1452: note = nucleotide variant of gene NCgl0885
  source 1..1452: mol_type = other DNA
atgcgtaaaggaatttcccgcgtcctctcggtagcggttgctagttctattggattcggttcggtgttgtctggaaccggcatcgcagcagctcaagactctgcatttgactacggtatggatccgagcatgaactacaacccgatcgacgacatcaaggatcgtccccaagggttatccaaccttccctacttcggaagcaaactaaccagctggggctcatcagatgccaccgcctcatccggcgtcgtgacctccgcgctcccgcagtacaccgatccgcgctaccccctcggcaaagacgacctgcccaaggcaaccatcgacatggagccagaagttcttgcgcgccttgagcgattcgtcggcgttgacggtgatcgcatccgccaaatcaacgcgtactcgccatcaatgggacgcaccattcctctagtctgggttgttccagaagacaacaccgtgcctggcccaacggtctacgcactcggcggcggcgacggtggccaaggcggccaaaactgggtcacccgcaccgaccttgatgagttgaccagtgaaaacaacatcaacctcatcatgcccatgctcggatcttttagtttctacgctgactgggcaggcgaaagcgaatccatgggtggtgcgcaacagtgggaaacattcctcatgcacgaactacccgagccgctagaagcggccatcggcgcagacgggcaacgcagcatcgtcggcatgtccatgtccgggggatcggtgctgaactttgcgacgcatgaccccaacttttattcctctgtcggctcattttctggatgtgccgaaaccaactcctggatggggcgccgtggcatcgcagccactgcctacaacggcaatgtcgtgcctgagcaaatctttggtgaagtagacagtgattactctcgctataacgatcctttgctcaacgctgcgaagctcgaagaacaagacaacctctacatcttcgccggttccggtgtgttctctgaactagatgtcatcggtgacaacgcaccgattgatgaggatgcgttcaaaaaccgcgtcttggttgggtttgaaatcgaagctatgtccaacacctgcacccataacctcaaggctgcgaccgatcaaatgggcatcgacaacatcaactacgatttccgaccaaccggaacccacgcctgggattactggaacgaagcgctccaccgcttcttcccgttgatgatgcagggcttcggcctcgacggtggtcccatcccgatctataaccctaacggtgtgacctccagcgagtcttcctcagaactgtcttctgatgtgagccttggcaccgtgatcggtagtgtggcgggaagctccggatcaagtgcaggcagcagcgtccgagagttcattgcaggaagttccggatcaagccaatcagcaggaagcttctacgaataa

SEQ ID NO: 26 - DNA, 3747 bp, synthetic construct
  misc_feature 1..3747: note = nucleotide variant of gene NCgl1142
  source 1..3747: mol_type = other DNA
atgactacaactacttcttctgggaagtcttctgaaaagatcaaccccctcttcaagctcggcagtttcctaagaaaaggcaccgtcggttctgaaggccagcagattttccttcagggcggacgccaagccgatgtgttttatcgcaaccgatgggctttcgataaagtcgtgcgctccacacatggcgtgaactgcacgggctcctgctcgtggaaagtgtatgtaaaagacggtgtgatcacctgggaatcccaggcagtggattacccaactaccggtgcggatatgcccgactatgaaccacgtggctgccctcgtggtgcatcattttcctggtacacctactccccaacccgcatccgctacccatacatccgtggcgtgctagttgatatgtaccgcgaagccaaggaacgcctgggcgatccggtgctggcgtggcgcgacattgtagaaaccccagaaaagcgcaaagcatatgtatcccagcggggcaaaggtggcctcatccgcgttcagtatgaggaagccatggagattgctgcggcagcccatgtgtacaccatccgccaatacggccccgaccgcattcatggattcaccgttattcccgcaatgtcgcaggtgtcttacggtgctggtactcgcttcttgcagatgatcggcggagtggcgctgtccttctacgattggtacgccgacctcccaccagcatcaccacaaactttcggcgatcaaactgacgttccggaatctggcgactggtacaactccagctacctcatgatgtggggttccaacattccggtgacccgcacgcctgactcccacttcatggtggaagcccgctacaagggcaccaaggttgttgtggtttccccggatttcgctgactccaccaaatttgctgatgaatgggcacgcatccaccctggtactgacggcgcactcgcctttgccatgggccatgtgatcttgaaggaattccatgttgacaagaagacgccgtacttcatggactacatgcgcaaatacacggactctcctttcctcgtggaattagatgagcacggcgatggcacctacaccccaggtaaattcctcactgcagaccgcgcagctgatatctccccagcgcttgccgccactccaaatgccacccaccgtctccttgtgctgcaaaaagatggctcagttgtagatcccggtggcactgtcgcggaccgttggggtgaagaaggcatgggtaagtggaatctgcgcttagacggcgtagatccagtgatgactattgcagatgtacagactgacaccgaaactgcggaagtcctcttcccccgcttcgatctcccagcaactgccacccaagaaggccccattggtgctggcaccatcagccggggcgttcccaccatcacgttgaatggccgaaagtacaccactgtctttgatgtgttgctcgcacactacggtgtgaaccgcgaagagctcaaccttcctggtgagtggcctaaggatttccaggatccagtcatgggtactcctgcgtggcaggaatagctcacgggtgttcctgctaatcaggcgattcgtttgggtcgggaatttgctcagaatgctgatgattccaagggccgttcccagatcatcatgggtgctggtgtgaaccactacttccatgcggattctatttatcgcacattcttggcgctgacctctatgtgtggcacccaaggtgttaacggtggcggttgggctcactacgttggtcaggagaaactccgtccaatgaatggttgggcacagtatgcctttgctacagactggcagcgtccaccacgtcagatgatcaccactggtttctactacctcaccacggatcagtggaggtatgacaacactcgtgctaatcgtctggcttccccactggctaatcgtggcaccgtgggtgacaaaatgacggcggataccttggtggaatccatgaaacgtggatggatgccgtcattcccgcaattcaaccgcaatcccctcatcttgagccaggaggcggaagaaaagggcgtgtctgtttctgaccatattgttcagcagctcaccgatggtgacttgcagttcgcctgcgaggatccggatgcaccggaaaactggccacgcattctgcttaactggcgcacaaacctaatgggctcttcagctaagggcacggagtttttcttgcgccatatgttgggtgtggattctgatgcatctgctgaagaaaacgcgccggaggatcgtccaagttccattgtgtggagggatgaggctccggaaggaaagctcgatttgatgctgaccacggatttccgcaacacttccaccaccttggtctcggatatcgtgctgccggcagccacctggtatgagaagcatgatttgtccaccacggatatgcaccccttcatccactcgttcaatgctgcgatcaacccaccgtgggagacgcgtactgactgggaggtcttccacgatctcaccaaagaattctcctcacaggcagcaacctggttgggcacccaaaccgatgtgatcaccgcaccgattgcccatgactccccggatgagctcaatatgcctggcggtatcgtgccagatattgatgaggtcgggctgatccctggcaagacgatggccaagatcatcccggtggaacgtgattactccaaggtgtatgaaaagtggacacacttgggaccactcaccgccaaagcgggtaccggaacccacggcactgcgtttaacgtgaccaagcaaaccgaggagctggcgctgatcaacggcacctccatcacggagtctgctggtgaacgcccccgacttgattccgcagtcaaggccattgagatgattctgcacttaagtggcgtgtctaatggtgaggttgccgccgaaggtttcaagaatcagggtgcacgcgtgggcaccgacatgatggatctgattgcagaccacgaaggtacccacatcaattgggacatggtcaaagaacgtcccgccgaggtgatcacctcaccggagtggactggttccaagaaggacggacgtcgctacaccgcgttttccatcaacattgaatacgacaagccgtggcacaccctgtctggtcgcatgcactactacctcgaccacgattggtttattgattacggcgagcagttgccaatctttaggccaccgttggacaagatccacatcaatggtgaggtcggccctggccagtcggtcacaggcaccgacggcgaaccagaagtaaccgtgcgttatctgaccacccacaacaagtggtcgattcactcgcagtactacgacaatctgcatgtgctttctatttctcgtggcggccaggtgatctggatgtccaacaaggatgcagagaaactcggtatcgctgacaacgattggatcgaggcttataaccgcaacggcgttgtttctgctcgtgcgattgtctcccaccgcattcctgaaggcaccgtgtttatgaaccacgcgcaggaacgcaccgctggcaccccgctgaacgagaagtctggcaggcgcggcggaactcacaactctcttactcgaatcatgattaagccggtccatgttgccggtggctacggccacttaacctatggcttcaactacatcggcccaaccggaaataaccgcgatgaggtcaccagaattcgtcgccgctcccaggaggtgcagtactaa

SEQ ID NO: 27 - DNA, 1452 bp, synthetic construct
  misc_feature 1..1452: note = nucleotide variant of gene NCgl1165
  source 1..1452: mol_type = other DNA
atgactacagctcttgaagagcagaacgcacagcaggcagccactgccggccgtgtcgtgcgtgtcattggtgcggtcgtcgacgtggagtttccccgcggcgagctgccagcactgtacaacgcacttactgtagaggtaaccctcgaatcagttaagaagaccgttgttctcgaggttgctcagcacctcggcgacaacctcatccgcaccatcgctatggcaccaaccgacggacttgtccgcggtgctgctgtaaccgatactgcacgcccaatttccgtaccagtgggcgatgttgttaagggccacgtattcaacgctttgggcgactgcctagacgacgtttccctgaacaacaacccagagatcgagcgttggggcatccaccgcgagccaccatcattcgatcagcttgagggtaagaccgagatcctggaaacaggcatcaaggttatcgaccttctcaccccttacgttaagggtggaaagatcggcctcttcggtggtgcaggtgtgggtaagaccgttcttatccaggaaatgatcacccgtattgcacgtgagttctccggtacttccgtgttcgcaggtgttggtgagcgtacccgtgagggcaccgacctcttcctcgaaatggaagaaatgggcgttctccaggacaccgccctggtgttcggtcagatggatgagccaccaggagtccgtatgcgcgtggctctgtccggcctgaccatggcggagtacttccgcgatgttcagaaccaggacgtgctgctgttcatcgacaacatcttccgtttcacccaggcaggttctgaggtttccacccttctgggtcgtatgccttccgccgtgggttaccagccaaccctggctgacgagatgggtgttctccaggagcgcattacctccaccaagggccgttcgattacctctctgcaggccgtttacgttcctgccgatgactacaccgacccggctccagcgaccaccttcgctcacttggatgcaaccaccgagcttgaccgctccattgcttccaagggtatttacccagcagtgaacccactgacctccacctctcgtattctcgagccagcaatcgttggtgagcgtcactacgaggtttctcagcgtgtcatcggcattctgcagaagaacaaggaacttcaggacatcatcgccatccttggtatggacgagctttctgaagaggacaagatcaccgttgcacgtgcgcgtcgcatcgagcgcttcctgggtcagaacttcttcgttgcagagaagttcaccggtcttcctggctcctacgtgccactgaccgacaccgtcgacgctttcgagcgtatttgcaacggcgacttcgaccactacccagagcaggctttcaacggcctcggtggtttggacgatgtcgaagctgcatacaagaagctgaccggaaagtaa

SEQ ID NO: 28 - DNA, 1764 bp, synthetic construct
  misc_feature 1..1764: note = nucleotide variant of gene NCgl1253
  source 1..1764: mol_type = other DNA
atgacgcctacccaaaatgagatccacccgaaacatagctactcccccatccgcaaggacggtctcgaggtcccggagaccgaaatccgcctcgatgactcgccaagcggccccaacgaacccttccgcatctaccgcacccgtggcccagaaaccaaccccaagcagggacttccgcggctgcgcgagtcatggatcaccgcccgcggcgacgttgccacctatcaggggcgcgagcgtttgcttatcgacgacggccgctcggcaatgcgtcgaggtcaagcttcggctgagtggaaaggccaaaaaccagctcctttgaaggcgctacctggcaaaagagtcacccaaatggcctatgcacgtgctggcgtgattactcgtgaaatggagtttgtagcgctgcgcgaacacgttgatgcggagtttgtgcgctctgaggtggcgcgcggtcgggccattattcccaacaacgtcaaccaccccgaatctgaaccgatgattattggtcgcaaatttttgaccaaaatcaacgccaatattggcaattctgcggtcacctcttcaatcgaggaagaggtgtccaagctgcagtgggccacgcgctggggtgccgataccgtgatggatctatccaccggcgatgatattcacaccacccgcgaatggattatccgcaactcccccgttcctatcggcaccgtcccgatctaccaagcgctggaaaaagtaaatggcgtggccgcagaccttaactgggaagtattccgcgataccatcattgagcagtgtgaacaaggcgtggactatatgaccatccacgccggcgtcctgctggcttatatcccactgactacccgtcgtgtcaccggcattgtctcccgcggcggatccattatggccggttggtgtccggcgcatcaccgcgaatcattcctctacgagcatttcgacgagctgtgcgaaatctttgcacaatatgacgtcgcattctccctcggtgatggcctacgccccggatcgcttgccgatgccaacgacgccgcgcaattcgccgagctgaaaaccattggtgagctcacccaacgcgcctgggaatacgatgtacaagtaatggtcgaaggacctggacacgtgccactaaacatgatccaggaaaacaacgagctggaacaaaagtgggcagcggacgcacctttttacactcttggaccactagttaccgacatcgctccaggttatgaccacatcacttctgccattggtgcagctcacatcgccatgggtggcaccgccatgctgtgttatgtcaccccgaaagaacaccttggcctgcccaaccgtgacgacgtcaaaaccggcgtaatcacctacaagctcgctgcccacgcagcagatgtggccaagggtcatcccggcgcgcgtgcctgggacgacgccatgagtaaagcgcgttttgaattccgttggaatgatcagtttgcgctctccctcgaccccgacactgcaatcgcttatcacgacgaaaccctgccggcagagcctgcgaaaaccgcacacttctgttcaatgtgtggcccgaagttctgctccatgcgaattagccaggacattcgcgatatgtttggcgatcaaatcgcggaattggggatgcctggggttggggattcttctagtgctgttgcttctagtggggcacgggaggggatggctgagaaatcccgggaatttattgctggtggtgcggaggtttatcggcgttag

SEQ ID NO: 29 - DNA, 2163 bp, synthetic construct
  misc_feature 1..2163: note = nucleotide variant of gene NCgl1315
  source 1..2163: mol_type = other DNA
ttgcttgcacgctgttttgctgcgggccgcaacgtgtccaccctgtggcgtatcctagaatgcatggcttttgctgctgaacatcctgtcctgtcccactctgagcaccgcccggttggtgaaatcgagcgtagcgatgacaaatttgttgtcgttagtgaatttgagcctgcgggtgaccagcctgcggctattaaagagctcgatgagcgcttggatcgcggtgagcgggacgtcgttttgatgggtgctactggtacgggtaagtccgcgactgcggcgtggttgatcgaaaagcagcagcgccccgctttggtgatggcgccgaataagacgctggctgcgcagttggctaatgaattgcggcagctgttgcccaataacgcggtggagtatttcgtgtcttattacgattactaccagccagaagcgtatatcgcgcagactgatacctatattgaaaaggactcctcgattaatgaggatgtggagcgtctgcgtcactcggcgacgtcgtctttgctgagtaggcgagacgtcgtggttgttagttcggtgtcgtgtatttatggcttgggcactccacagtcttatcttgaccgttccgttgtgttgaacgtgggggaggagatcgaccgcgatcgctttttgcgcctattggtagatattcaatacgaacgcaatgatgtgggctttactcgtggtgctttccgcgtgaagggcgataccgtggacatcatcccggcctatggggaattggcggtgcgcattgagtttttcggtgatgaaattgatgcgttgtactacatccatcccctgactggtgacaccatccggcaggtgaatgagatccgtattttcccagctacgcactatgttgcgggacctgagcggatggaaaaggcagtcgctgatattaaggcggagttggaagtgcgcctggctgatttggagaaccgtggcaagttattggaagcgcagcgtcttaggatgcgtactgaatatgacttagaaatgatcgagcaggttggtttctgttcgggcattgagaactattctcgccacattgatggacgtggggagggaaccgcaccggccacgctgattgactatttcccagaggatttcctcaccatcatcgatgagtctcacgtgacagtcccgcagatcggcggcatgtttgagggcgatatgtcccgtaaacgtaacctcgtagaattcggtttccgcctgccatccgcgatggataaccgcccattgacctgggaggagttcgatgaacgccgtggccaaacggtgttcatgtctgcaactccaggcaagtttgagatcgctgctgctgatggtgagtttgtggagcaggtcattcgcccaacaggtctggtggatccaaaggtcaccgtcaagccaacgaaggggcagattgatgatctgatccatgaaattcgccaacgcaccgataaagatgagcgcgttttggtcaccacattgaccaagaaaatggctgaggatcttactgattacctgctggaaaacggcatccgcgtgcgctacctgcactcagatattgataccttgcagcgtgtggaattgctgcgtcagcttcgcctgggcgaatacgatgtgttggtaggtattaacctgctgcgtgagggccttgacctgccagaagtctctctggttgcgattctcgacgccgacaaggaaggcttcctgcgctccaccacctcactgattcagaccattggccgcgccgcccgaaatgtgtccggcgaggtcatcatgtacgccgacaagatcactgattcgatgcagtatgccatcgaggaaaccgatcgacgccgtgaaaagcaggtcgcttataacaaggaacacggcatcgatccgcagccgcttcgaaagaaaatcgcggacatcctcgaccaggtctatgacaattccgctgatggagcaggaccttctgcctctggcgatgcggcagtcgtggctaaacctgacgtgtctagcatgcccgccaaagaagtgcaaaagcttatcgacgacctcagcgctcagatggctgcggccgcgcgggagctcaagttcgagctggcagggcgtctgcgagatgagatcttcgagctcaagaaggaactgagaggtatcaaggatgccggcatctaa

SEQ ID NO: 30 - DNA, 972 bp, synthetic construct
  misc_feature 1..972: note = nucleotide variant of gene NCgl1511
  source 1..972: mol_type = other DNA
atgggtgatttgaaaatgcaacgttctggaggagaacccttggacacgatcaaggcctatattgcgctaacgaagcccagggttattgaactcctccttgtcgccacaatccccacaatgcttcaggctgaacgcggtgagaacaacattgtgctcatcttgctgactgtgttcggtggctggatgggtgcggccgccgccaacaccttcaacatggtggcagactccgatattgatcagcgcatgggacgcactagggctcgccctttggtgcgccacaccgtgagtaatcgcgacgcctccatttttgcgtgggtcctgacagtggccagcttcttgtggctgtggctgctgtgcgattcgatgctcgccggcatcttcgtgttgatcacgattttcttctacatttttgtctacaccaagtggctgaagcgccgcacgcacatgaatatcgtgtggggcggagccgcaggttgtatgccagtgctcgtcggctgggcagtgatcgttgatcagtttgagccaggcgttccacagcagtggtggcaggcaattgtcctgttcatggtgattttcttctggaccccacctcacacctgggctctggccatgaagtaccgcgaagactacaaggcggctggcgtcccaatgcttcctgtcgtgcgcaccccagtccaggtcaccgcacaaatcgtgtggtactccgtggcaactgtgctgaccaccttcttgctcatcccagcaactggttggatctacgcagcgatcgccgtcatttccggcgtcaccttcttgttcatggccatcaagctgcacctcggcatcaaaaacggtggcaaggtcaagcctctgaagctgtttattttgtccaacaactacttggcagtcctcttcgtggcattgtccgtcgacgcggtcctcggccttgagaccatcggcgagatgctcggctggaccaccaccttcttctaa

SEQ ID NO: 31 - DNA, 558 bp, synthetic construct
  misc_feature 1..558: note = nucleotide variant of gene NCgl1588
  source 1..558: mol_type = other DNA
atgaagcttttctcccgcacctcactggttgcacttggtaccgctgcagctatcactctctccggcgtaaccgctcctgcattcgctgatgaggactccaacgcagctgtaagtgctcttaagaccgctgaagataatacccctgaggcgccaggggcttctactcccctgaagcttgagcagcctggcaccatcaccggcgtccctggcaaggcgatcaccccggtcactgttaaggtcatcgcaggcgaagcagaatccttcacctcagacaaccttccttctggtctccttatcgacaacaccggaaagatcaccggtactccaaagaaggaattcactggttccgcaaagatcattgccaagaacgaagcaggcgttgaagcagaagtttacgttaactttgatttcaacgaagagccttccagcgaagagccttccagcggttcttccgacactgacaacatcgaaaactggatcaagatcatcacagcagtcatcggtgcactaaccaccattttaaccttcagtaccaagctggattccttcctgaagtaa

SEQ ID NO: 32 - DNA, 1587 bp, synthetic construct
  misc_feature 1..1587: note = nucleotide variant of gene NCgl1815
  source 1..1587: mol_type = other DNA
atgcgctcagatgtcatcgagttaccggagggggtgagcaaggacgaagctgatcaggtggaggttgcggaagcgcgacttaatgagggcgcacgattgatggctgcaactgggtgtgaggctatgtggccaacaggtttctcagtttgtggccggattcttgacgcttatcggcaggttggaggtcagttgtcatggcttgggccaccgaagtcaaacgagttgaccaatcccgacggtgttggcaaaagaagtgaattttttggtggagccatctattggcacccagacacaggcgcttatgcagtgaccttggacggtttgcgacagtgggggaccttgaactgggaatcagggccattggggtacccaacctctggtccgatggatacaaactatccccttactcagcgacagacttttcaaggtggtgacaactactacaacccattgactggcggtgctgtgtggggcgatattaaacagcgctacgaagaacttggcggctcgaatcatgccattggcatcccgatcactaatgagctacctagcggtactgagtatttttacaataatttctccaatggaacaatttcgtggcgaaatgatcgtcagacacggtttatgtatttggctacgcagcgggtgtgggatgcgttgggtcgggagacgggtcgtttaggttttcctgaagcagatgaaacacctgaggtttctggtctattccatgtggtgaattttgcggagcgcggggtgattgcgtggaatggaatcctaggcgccagagagctgtatggtgatgtttactccctgtggctgcaataccaaaataccgatactcctttagggtggccgataccatcattgacatcattaaatgagtcactcgaacaagaattcaccagaggtgttgttttaggctcaggtgatgcactgacatggattcctgacgatgaagaaagaagtttggaggatttcctcccaattggaagtagcggctcatcctcatcgagccaagagatgaccctgttttcccagcgtgcacaatacgtggattgcaagaatcttcccgatttagatgagcagagaaaaactgaaaacaacattgaaaagaatggtggcccgatcaaaaaagagtatagttcgcgaggtttccccaccgagttcagatttgtggtgagaaaagggcattatgaccgttacaggaatgaaggctggggatatttaaaaaactattgcaaacacaacttcgccaaccacgctatggctgaggccgtagtagataaagcggtgattgattatggctcatcgccaggaaccagctattacaagttcgagaaaacggtgtactttctagattgcagaacttatacattcaataagaactcaggatgtaaagaaatgcacgctccgcaatgggtgactattatttacaatcctcatactttcactggagcaaattcgaacagacccaagggggtaatttcagcatggtgtaattcaaccccacctggtggaatcgaacacgagccggaaatttcccaatgtcctgatcatgtgaatctttataataagcttcgcatatga

SEQ ID NO: 33 - DNA, 795 bp, synthetic construct
  misc_feature 1..795: note = nucleotide variant of gene NCgl1859
  source 1..795: mol_type = other DNA
atggtcagccaaacggaaagacagcatgcaattgcttctttactggcaccaactggtgcggtgtctgtaggagatttagccgagcatttccatgtgacaaccgaaacagtgcgacgtgatcttcggatcatggagtcactgggtttgttgcaacgagttcacggtggcgccattagcccagagcccatgggtacgtctccccctcggctgaaacctgccttggttaaaggaatgccaccggaaccccgtgttttagaacttgcagaaactgcagtttccctcatcacacctctagcacgcagcattttcctggattcaggtttagcgtgcacggcgattgccacggtgttgggggatcctccagaagatgccaggtggactgttgttacaagttcccccggcgctgtgattgccttgtccgcgacagatgccacctccacggtggtgctgcacgggcaggttcacggtaattgttcttcaatcattgggtccacggcagtagacatgatttcgcagttgcgcgctgatatcgccttcgtggaggttgatgcgattcaatccgatacaagtctgtgcacgtttttcccggagacgattcccatcaagcaagccatgatcaaaaacgcggctttcacagttgctgttctcagcccgagatctccccaagatcaagaacttcaacttttgaagcaccctttttccaccttggctgattttgatgcccttgttaccgatgaccacacgctagattttccagttttgcccgaccacaactttcaggtggtaaccccatga

SEQ ID NO: 34 - DNA, 1581 bp, synthetic construct
  misc_feature 1..1581: note = nucleotide variant of gene NCgl1874
  source 1..1581: mol_type = other DNA
gtgacgcagcaattgaaccacgcaaaggtaaatcaacatcccggtcaagccaccctcccagaaaccgcagaggggcaggttcgcacctacgaggtaaaaacctacggctgtcagatgaatgtgcacgattctgagcgcctttcgggcctgctcgaggaggctggatacgttgctgctccggaggacaccactccggatcttgtcgtatttaatacgtgcgccgtgcgtgaaaacgccgatatgcgcctctatggcactttgggcaacctgcgcagcgtgaaagaaaagaacccaggcatgcaaatcgctgtcggtggttgtttggctcaaaaagacaaagataccgtggtgaaaaaagcaccgtgggtggacgtggtgtttggtacccacaacattggttccttgccaaccttgcttcagcgcgcggagcacaatgcccaagcggaagtcgaaattgtcgattccctcgagcagttcccgtcagtacttcctgcaaagcgcgagtctgcttacgctggttgggtgtccgtatcagtcggatgtaacaacacctgtactttctgcatcgttccgtcgctgcgcggtaaagagcaggaccgtcgaccaggagacatcctcgcagaggtacaagcactggtggatcagggagttaccgaggtaactctacttggccaaaacgtaaatgcttacggcgtgaactttgttgatcctgagctagagcgcgatcgcagtgcattttccaagctgcttcgtgcctgtggtgagatcgaaggcctcgagcgggttcgcttcaccagccctcaccctgcagaattcacctctgatgtcattgacgccatggcagagaccccaaacatctgcccgcagctgcacatgccactgcagtccggatctgacaaggtgctcaaagagatgcgccgttcctaccgatccaagaagttcctctccatcttggatgaggtccgtgcgaagatccctcacgcctctatcaccaccgatattattgtcggattccctggcgaaacagaggaggatttccaagcaaccctcgacgttgtcaagaaggcacgctttacttctgcttacaccttccaatacagcccacgccctggcacccctgcagcggaatatgaaaaccagcttccaaaagaagttgtgcaggaacgctacgagcgcctcatggtcgttcaggaacaagtctgcgaagaagaaaaccaaaagctcatcggcaccaccgtcgaattgctggtccaggctggcggaggccgcaagaacgatgccaccaagcgcatgagtggtcgcgcacgcgatggacgcctcgtgcactttgcgccagagggcgacattgatggtgagatccgccccggcgattttgtcactgtcacggtgactgaggccaagcctttcttcctcatcgcagactccggtgtgcagacccaccgccgcaccaaagctggtgacaactctgcagttggtcaagttccaaccacagcaccgatcggtgtgggcttgggactgccacaaatcggcgcaccaaaggtggctcctgccacagaatctgcctgctgctccattaactaa

SEQ ID NO: 35 - DNA, 975 bp, synthetic construct
  misc_feature 1..975: note = nucleotide variant of gene NCgl2245
  source 1..975: mol_type = other DNA
gtgtccaaaacagaagaaggccgttcagcggccataattatttacgcgtttccaactttcattctgctgggcgcgatcattgcgtttatcttcccggaaccattcattccgctgacaaactacattaatatcttcctcacgatcatcatgttcaccatgggtttgaccttgacggtgcccgattttcagatggtgcttaaacgtccactgcctatcttgatcggtgtagtagcgcagtttgtcatcatgccattcctggcgatcgtggttgcgaaaatgttcaacctcaacccagcactcgccgttggccttctcatgctgggatccgttccgggtggcacctcctccaatgtgattgcgtttctcgcccgaggagatgtcgcgctatcggtcaccatgacctctgtgtccaccattgtttccccaatcatgacgcctttcctcatgctcatgctggcaggtactgaaaccgccgtcgatggtggaggcatggcgtggactttggtacaaacagtgctgctgcctgtgatcatcggcctagttctgcgtgtcttcttgaacaagtggatcgacaagattttgccgatccttccttatctctccatcctcggtatcggtggcgtggtgttcggcgcagtcgcagccaacgcggaacgactcgtgtctgtcggactcatcgtgttcgttgcagttatcgtgcacaacgtacttggatacgttgtgggatacctcaccggccgtgtattcaaattcccagaagcagcaaaccgcaccatggcgattgaaatcggaacccaatcctcaggcctcgcatcgggaatggcaggacgattcttcaccccagaagcagcccttccaggtgctgtcgctgccttggtccacaacatcaccggcgcagtttatgttgggctggtacgaaacaggcctttgactaaggcatcaaggaagaaggaatccgtcgcggtttccagctaa

SEQ ID NO: 36 - DNA, 882 bp, synthetic construct
  misc_feature 1..882: note = nucleotide variant of gene NCgl2580
  source 1..882: mol_type = other DNA
atgtcatttacagcttttcaaacagccctgctcgtgtggtttagagcaaatgcccgcgatcttgcgtggcgtgatcccaatacttcagcatggggaattctcctttcagaggtgatgagccaacaaactcccgtcgcgcgagtcgagccgatttggcgtgagtggatggaaaaatggcccactccggaagatttcgcgaatgcgagcaccgatgagattttgcggtcgtggggcaagttgggctatccacgtagggcgctgaggttgaaggaatgtgcggaggtgatcgtcgaaaagcatgccggcgaggtgccggatacggtggaggcgctgctcgcgttgccggggatcggtgattacacggcgcgcgcggtcgcggcgtttcattttgggcagcgcgtgccggtggtcgatacgaacgtgcgtcgcgtgtaccagcgcgcggtagccggacgttaccttgcggggcctgcgaaaaagcaagagcttatcgacgtctcccttctccttcccaacactcacgccccagaattctctgccgcaataatggagttgggtgctcttatctgcacggccacttccccaaagtgtgacacctgcccactgcttgaccagtgtcaatggcaaaaacttggctgtccctccccgagtgaagaggagctggcttcagcgaaaaagcgtgtgcagaaatttgtgggaaccgaccgacaagtccgcggcctgatcatggacgtgctgcgcaatgccaccgcacctgtgccactatccgcgattgatgtcgtgtggcctgacgatgcccaacgctcccgggcgctgttttcgctcattgaggacggactcgcggaacaagatgaggcgggttatttccacctgccacgataa

SEQ ID NO: 37 - DNA, 2682 bp, synthetic construct
  misc_feature 1..2682: note = nucleotide variant of gene NCgl2629
  source 1..2682: mol_type = other DNA
atggtgaacacgttgaactctaaaaccgtgaatgtaccccgttttgccagaggcgttgttgctgcagccacagcgctattttttggcgctttggtaagcctcgcgcctagtgcgttggcgcaggaaccacctgcagttgaggccggagcgtcaggttctttgagcaacctgggtgcctgcatcgctgataaaggcactcttgatgtcatcatcatgatcgatgagacagaatccttgatccatgaagctcgtgacggcgtggtcaacgccaatgaaccaggcgcggacgcacagcaccaccgtgttcctgcagcacagagctttgtggatgagcttctagccaagcaaagcgatggtgatctgaacacccgcatccgtgttgctggtttcggccagacgtacaaatctggtgccactgatccagacaattacggagcatggacgcaactagatgcctccaccgttggcggagtacaagatgaaatctcccgcttcgctgaccgcacccaggagcagtacaccaactacgcctccgcgattgagggcgcttaccaggacttcactaggtccggctctgaggacgcctgccgcatgctggtgaccttcaccgacggcgcactgaccgctcaagaaggcgccgatgttgcagaagcagcactgtgcgcgccgggtggcgtcaccgatcgactgcgcagtgctggcatcacccacatcggcatcggtttatcggcacctaccaacccatctgatttcagcctgctgcgcggaaccaccgcaggtggcggaacatgtggtgtcgaaccagctaacggtgcattcttcccagcagataacgtgggcggacttttcgcagcattccgtgaagcccttgcgattggtggtgaaacaattggtgaaacccgagctggtgatcctttcagcttcaccctggacaactcggtgaactctgtgcgtttcaccgcgatcgccaaggatgatctcggcccgaacgcccacttggtgctcaccgcacccaacggcgaaacggttgagctcaaagattctggaagcagcgtcgccaacagcactgacgtgagttgggaagccgaaagcagcccagtaaaaatggctgatggttccctcaacctgcagcaaggtggggattggaagggtgtctggcagattcagttccaaggaattgatcctgcagcggttgatggacgcgtattcaactcagtggagatccagcctgacctccagcttgtgttcagtggcggtgattcgacgtcaggtgcacttaaccttcgcgatgatcagcagctgaatatgcagctggtgggccgtgatggtcagccacgcatccttgaggggtccgcgctggtcgatcttggtttcacccgcgcagataccggcgagttcgcccctttggctcaaggaattgatatttctggcggcgaattaagcttcccgctggatacgatttcgcagctcccagccatcggcacggtggaagcgcgtaccacgatcaccaccgcaggcgtcgatgatctccccggcaccacgttgagcccaattctcaacaccacgcgcatcaccatcactcagcgcgatatgcctcagctgccagcgtcggttcgcttcacagcggatgaggacgttgttaccgtagacatccccatcaccggccccggcaaggtatggattgcaccgggaacccagctcagcggagtgcttccagacggcgtggacggcattgcagcatcaagtactttcgacagcccagataatgctttggtgctcggactggatgagcagggcacgattcctgttgaactaaccgtgagcgatcttcgtgacggactggtcaacggctcgattccactccagatctccaacgctgagggcgccaatgaaaccagcgtggatctgccgacagaaggcacgttgagcgttcccattaacgcctccactttcgcattggcattcattttggcccttgtgctttccctcctgattccgctgctcattttgtatattgtgcgtttcctctccgcaaaggttccgtcctctgcgatgagtggcgtgcgcattccagtggaattctccggtgaagctctgcgctatgcgggcagcactatgcctgatctcgcatcgcaaaccaccgccaccaagcaggtcgttgttcatggagacaccttcaatgtggaaggccacaaacttaaagtccagcgcttccagctgaacccgattgcgtctcctgcagtgatcgtgcagaccgacccgtcgatcagcttcgacggcaaacaaaagggcacacaagctaaactcccgctggcggtccaaggcagttggttcctcactgcaagcggcgctgacccttccaagatggaactcatcgccctgacaaacctgccgctcgagcagggccaaatcgaccgcatgatcgcaggtatcaccagcaaagcccctgatagggcacgcgaactacaaaaattgcttgacgacgccgcgacctcccagcccgcaaaggttccaccgcgcgccccagccgcgcagggccacgtcgaaaagcaagctcctagttttggcactggttccggtggtgttttcggctccagcaatggtggaggctttggctccggtagcggatccaacgacacaaatggtggatttggttccagcggcggcttcggcgcgcgataa

SEQ ID NO: 38 - DNA, 723 bp, synthetic construct
  misc_feature 1..723: note = nucleotide variant of gene NCgl2863
  source 1..723: mol_type = other DNA
atggctgaccgcacaccgaccaccgccacgcccccggggtgggtgctggtcgtcgatgatgaacaacccctggctcagatggtggcctcctacctcatccgggccggcttcgacacccgccaggcgcacaccggcacccaggccgtggacgaggcccgtcgcttttcccccgatgttgtggtgctggatctggggctgcccgaactcgacggcctggaggtgtgccgacggatccgcaccttctcggactgctacatcctcatgctcaccgcgcgtggcagcgaggacgacaagatcagcggtttgaccctgggggcggatgactacatcaccaaaccttttagcatccgggaactggtgacccgggtgcatgcggtgctgcgccgcccgcgcaccagcaccaccccaccgcaggtgaccacccccttgatcgttggtgacctcatccttgaccccgtcgcccatcaggtgtgggtgggggagacgaccgtggagctcacccgcacggagttcgagctgctggttgccctggccctgcgccccggccaggtgctgacccgccacgacctgatcaccgaggtctgggacaccacctgggtcggcgatgaacgcatcgtcgatgtccacatcggcaacttgcgtcgcaagctcggcaccgacacccggggccgggggtttatcgacaccgtgcgtggcgtgggctaccgggtggggcagccatga

SEQ ID NO: 39 - DNA, 40 bp, synthetic construct
  misc_feature 1..40: note = NCgl0337*_F
  source 1..40: mol_type = other DNA
tgaattcgagctcggtaccctttcgtgcgttacgtactaa

SEQ ID NO: 40 - DNA, 40 bp, synthetic construct
  misc_feature 1..40: note = NCgl0337*_R
  source 1..40: mol_type = other DNA
gtcgactctagaggatccccctattgctcattgttggcct

SEQ ID NO: 41 - DNA, 40 bp, synthetic construct
  misc_feature 1..40: note = NCgl0658*_F
  source 1..40: mol_type = other DNA
tgaattcgagctcggtacccacggacccaagcaagacctc

SEQ ID NO: 42 - DNA, 40 bp, synthetic construct
  misc_feature 1..40: note = NCgl0658*_R
  source 1..40: mol_type = other DNA
gtcgactctagaggatccccagatcgcactcaacggtttc

SEQ ID NO: 43 - DNA, 40 bp, synthetic construct
  misc_feature 1..40: note = NCgl0674*_F
  source 1..40: mol_type = other DNA
tgaattcgagctcggtaccctgctgctgtctggctatttc

SEQ ID NO: 44 - DNA, 40 bp, synthetic construct
  misc_feature 1..40: note = NCgl0674*_R
  source 1..40: mol_type = other DNA
gtcgactctagaggatccccccaaggatgactaagcaagc

SEQ ID NO: 45 - DNA, 40 bp, synthetic construct
  misc_feature 1..40: note = NCgl0686*_F
  source 1..40: mol_type = other DNA
tgaattcgagctcggtacccgcccacgcattatttccgga

SEQ ID NO: 46 - DNA, 40 bp, synthetic construct
  misc_feature 1..40: note = NCgl0686*_R
  source 1..40: mol_type = other DNA
gtcgactctagaggatcccccagaccactggaacgctgac

SEQ ID NO: 47 - DNA, 40 bp, synthetic construct
  misc_feature 1..40: note = NCgl0706*_F
  source 1..40: mol_type = other DNA
tgaattcgagctcggtacccggtgcggcccctgcaaaatg

SEQ ID NO: 48 - DNA, 40 bp, synthetic construct
  misc_feature 1..40: note = NCgl0706*_R
  source 1..40: mol_type = other DNA
gtcgactctagaggatccccggctacttctgcgatcctcg

SEQ ID NO: 49 - DNA, 40 bp, synthetic construct
  misc_feature 1..40: note = NCgl0885*_F
  source 1..40: mol_type = other DNA
tgaattcgagctcggtacccggaaactatggggattttgg

SEQ ID NO: 50 - DNA, 40 bp, synthetic construct
  misc_feature 1..40: note = NCgl0885*_R
  source 1..40: mol_type = other DNA
gtcgactctagaggatccccgcggctcgggtagttcgtgc

SEQ ID NO: 51 - DNA, 40 bp, synthetic construct
  misc_feature 1..40: note = NCgl1142*_F
  source 1..40: mol_type = other DNA
tgaattcgagctcggtacccttagcacgagtgttgtcata

SEQ ID NO: 52 - DNA, 40 bp, synthetic construct
  misc_feature 1..40: note = NCgl1142*_R
  source 1..40: mol_type = other DNA
gtcgactctagaggatccccggcactgtcgcggaccgttg

SEQ ID NO: 53 - DNA, 40 bp, synthetic construct
  misc_feature 1..40: note = NCgl1165*_F
  source 1..40: mol_type = other DNA
tgaattcgagctcggtacccgctccattgcttccaagggt

SEQ ID NO: 54 - DNA, 40 bp, synthetic construct
  misc_feature 1..40: note = NCgl1165*_R
  source 1..40: mol_type = other DNA
gtcgactctagaggatcccctcattcgcccagacggcgaa

SEQ ID NO: 55 - DNA, 40 bp, synthetic construct
  misc_feature 1..40: note = NCgl1253*_F
  source 1..40: mol_type = other DNA
tgaattcgagctcggtacccaccaatggcagaagtgatgt

SEQ ID NO: 56 - DNA, 40 bp, synthetic construct
  misc_feature 1..40: note = NCgl1253*_R
  source 1..40: mol_type = other DNA
gtcgactctagaggatcccccaatcgaggaagaggtgtcc

SEQ ID NO: 57 - DNA, 40 bp, synthetic construct
  misc_feature 1..40: note = NCgl1315*_F
  source 1..40: mol_type = other DNA
tgaattcgagctcggtacccgtgtcttattacgattacta

SEQ ID NO: 58 - DNA, 40 bp, synthetic construct
  misc_feature 1..40: note = NCgl1315*_R
  source 1..40: mol_type = other DNA
gtcgactctagaggatcccccgtggccggtgcggttccct

SEQ ID NO: 59 - DNA, 40 bp, synthetic construct
  misc_feature 1..40: note = NCgl1511*_F
  source 1..40: mol_type = other DNA
tgaattcgagctcggtaccccacagcagccacagccacaa

SEQ ID NO: 60 - DNA, 40 bp, synthetic construct
  misc_feature 1..40: note = NCgl1511*_R
  source 1..40: mol_type = other DNA
gtcgactctagaggatccccataggcgatagcatggcaag

SEQ ID NO: 61 - DNA, 40 bp, synthetic construct
  misc_feature 1..40: note = NCgl1588*_F
  source 1..40: mol_type = other DNA
tgaattcgagctcggtaccctcacttaaataacatcttgc

SEQ ID NO: 62 - DNA, 40 bp, synthetic construct
  misc_feature 1..40: note = NCgl1588*_R
  source 1..40: mol_type = other DNA
gtcgactctagaggatcccctcacaaaggattagtcgcgt

SEQ ID NO: 63 - DNA, 40 bp, synthetic construct
  misc_feature 1..40: note = NCgl1815*_F
  source 1..40: mol_type = other DNA
tgaattcgagctcggtacccatttgcccgggagggcctaa

SEQ ID NO: 64 - DNA, 40 bp, synthetic construct
  misc_feature 1..40: note = NCgl1815*_R
  source 1..40: mol_type = other DNA
gtcgactctagaggatcccctgatcgggatgccaatggca

SEQ ID NO: 65 - DNA, 40 bp, synthetic construct
  misc_feature 1..40: note = NCgl1859*_F
  source 1..40: mol_type = other DNA
tgaattcgagctcggtaccccacttttaataacttcatac

SEQ ID NO: 66 - DNA, 40 bp, synthetic construct
  misc_feature 1..40: note = NCgl1859*_R
  source 1..40: mol_type = other DNA
gtcgactctagaggatcccccagacttgtatcggattgaa

SEQ ID NO: 67 - DNA, 40 bp, synthetic construct
  misc_feature 1..40: note = NCgl1874*_F
  source 1..40: mol_type = other DNA
tgaattcgagctcggtaccccaatgacatcagaggtgaat

SEQ ID NO: 68 - DNA, 40 bp, synthetic construct
  misc_feature 1..40: note = NCgl1874*_R
  source 1..40: mol_type = other DNA
gtcgactctagaggatccccttcgggcctgctcgaggagg

SEQ ID NO: 69 - DNA, 40 bp, synthetic construct
  misc_feature 1..40: note = NCgl2245*_F
  source 1..40: mol_type = other DNA
tgaattcgagctcggtacccaatgcccacgaaactgaaaa

SEQ ID NO: 70 - DNA, 40 bp, synthetic construct
  misc_feature 1..40: note = NCgl2245*_R
  source 1..40: mol_type = other DNA
gtcgactctagaggatccccgctggcaggtactgaaaccg

SEQ ID NO: 71 - DNA, 40 bp, synthetic construct
  misc_feature 1..40: note = NCgl2580*_F
  source 1..40: mol_type = other DNA
tgaattcgagctcggtaccccccttctccttcccaacact

SEQ ID NO: 72 - DNA, 40 bp, synthetic construct
  misc_feature 1..40: note = NCgl2580*_R
  source 1..40: mol_type = other DNA
gtcgactctagaggatcccccttgggcagacaactacatt

SEQ ID NO: 73 - DNA, 40 bp, synthetic construct
  misc_feature 1..40: note = NCgl2629*_F
  source 1..40: mol_type = other DNA
tgaattcgagctcggtaccctggaacattcggaaggttcg

SEQ ID NO: 74 - DNA, 41 bp, synthetic construct
  misc_feature 1..41: note = NCgl2629*_R
  source 1..41: mol_type = other DNA
gtcgactctagaggatccccctcctgcagtgatcgtgcaga

SEQ ID NO: 75 - DNA, 40 bp, synthetic construct
  misc_feature 1..40: note = NCgl2863*_F
  source 1..40: mol_type = other DNA
tgaattcgagctcggtaccccgggcggcgcagcaccgcat

SEQ ID NO: 76 - DNA, 40 bp, synthetic construct
  misc_feature 1..40: note = NCgl2863*_R
  source 1..40: mol_type = other DNA
gtcgactctagaggatccccgaaatcaaaaaccctgctca

SEQ ID NO: 77 - DNA, 18 bp, synthetic construct
  misc_feature 1..18: note = NCgl0337_F
  source 1..18: mol_type = other DNA
caatgcagtgggggagag

SEQ ID NO: 78 - DNA, 18 bp, synthetic construct
  misc_feature 1..18: note = NCgl0337_R
  source 1..18: mol_type = other DNA
acagtgaaaaccttacgg

SEQ ID NO: 79 - DNA, 19 bp, synthetic construct
  misc_feature 1..19: note = NCgl0658_F
  source 1..19: mol_type = other DNA
atcaacgccggctatgcgc

SEQ ID NO: 80 - DNA, 18 bp, synthetic construct
  misc_feature 1..18: note = NCgl0658_R
  source 1..18: mol_type = other DNA
cgtcttcggtgcgggtga

SEQ ID NO: 81 - DNA, 18 bp, synthetic construct
  misc_feature 1..18: note = NCgl0674_F
  source 1..18: mol_type = other DNA
acaccaatgggctgtcag

SEQ ID NO: 82 - DNA, 18 bp, synthetic construct
  misc_feature 1..18: note = NCgl0674_R
  source 1..18: mol_type = other DNA
actcgttggtagagcacc

SEQ ID NO: 83 - DNA, 19 bp, synthetic construct
  misc_feature 1..19: note = NCgl0686_F
  source 1..19: mol_type = other DNA
gccgttcgtattctcggtg

SEQ ID NO: 84 - DNA, 18 bp, synthetic construct
  misc_feature 1..18: note = NCgl0686_R
  source 1..18: mol_type = other DNA
actcagcaattgggcgca

SEQ ID NO: 85 - DNA, 18 bp, synthetic construct
  misc_feature 1..18: note = NCgl0706_F
  source 1..18: mol_type = other DNA
ttgaacgtgatgcagcgc

SEQ ID NO: 86 - DNA, 18 bp, synthetic construct
  misc_feature 1..18: note = NCgl0706_R
  source 1..18: mol_type = other DNA
tagccattaatgatgccg

SEQ ID NO: 87 - DNA, 18 bp, synthetic construct
  misc_feature 1..18: note = NCgl0885_F
  source 1..18: mol_type = other DNA
ccatcgcgcaacggggcg

SEQ ID NO: 88 - DNA, 18 bp, synthetic construct
  misc_feature 1..18: note = NCgl0885_R
  source 1..18: mol_type = other DNA
cacaccggaaccggcgaa

SEQ ID NO: 89 - DNA, 18 bp, synthetic construct
  misc_feature 1..18: note = NCgl1142_F
  source 1..18: mol_type = other DNA
cttcagcagatgcatcag

SEQ ID NO: 90 - DNA, 18 bp, synthetic construct
  misc_feature 1..18: note = NCgl1142_R
  source 1..18: mol_type = other DNA
tgactccaccaaatttgc

SEQ ID NO: 91 - DNA, 18 bp, synthetic construct
  misc_feature 1..18: note = NCgl1165_F
  source 1..18: mol_type = other DNA
gcgcgtggctctgtccgg

SEQ ID NO: 92 - DNA, 18 bp, synthetic construct
  misc_feature 1..18: note = NCgl1165_R
  source 1..18: mol_type = other DNA
ttttgagtccttcctgcg

SEQ ID NO: 93 - DNA, 18 bp, synthetic construct
  misc_feature 1..18: note = NCgl1253_F
  source 1..18: mol_type = other DNA
ccgcgatttgatcgccaa

SEQ ID NO: 94 - DNA, 18 bp, synthetic construct
  misc_feature 1..18: note = NCgl1253_R
  source 1..18: mol_type = other DNA
gcgcgagtcatggatcac

SEQ ID NO: 95 - DNA, 18 bp, synthetic construct
  misc_feature 1..18: note = NCgl1315_F
  source 1..18: mol_type = other DNA
gaatgcatggcttttgct

SEQ ID NO: 96 - DNA, 18 bp, synthetic construct
  misc_feature 1..18: note = NCgl1315_R
  source 1..18: mol_type = other DNA
gatcagatcatcaatctg

SEQ ID NO: 97 - DNA, 18 bp, synthetic construct
  misc_feature 1..18: note = NCgl1511_F
  source 1..18: mol_type = other DNA
atgagcaagaaggtggtc

SEQ ID NO: 98 - DNA, 18 bp, synthetic construct
  misc_feature 1..18: note = NCgl1511_R
  source 1..18: mol_type = other DNA
taattggttcaaatttgg

SEQ ID NO: 99 - DNA, 18 bp, synthetic construct
  misc_feature 1..18: note = NCgl1588_F
  source 1..18: mol_type = other DNA
tactatttctgctgctgg

SEQ ID NO: 100 - DNA, 18 bp, synthetic construct
  misc_feature 1..18: note = NCgl1588_R
  source 1..18: mol_type = other DNA
tcttctacggtgtcagcc

SEQ ID NO: 101 - DNA, 20 bp, synthetic construct
  misc_feature 1..20: note = NCgl1815_F
  source 1..20: mol_type = other DNA
gtacgtggcgggggtaatac

SEQ ID NO: 102 - DNA, 20 bp, synthetic construct
  misc_feature 1..20: note = NCgl1815_R
  source 1..20: mol_type = other DNA
cccacacccgctgcgtagcc

SEQ ID NO: 103 - DNA, 18 bp, synthetic construct
  misc_feature 1..18: note = NCgl1859_F
  source 1..18: mol_type = other DNA
cacggttttcttcggcga

SEQ ID NO: 104 - DNA, 18 bp, synthetic construct
  misc_feature 1..18: note = NCgl1859_R
  source 1..18: mol_type = other DNA
agcggtgacggaatcaag

SEQ ID NO: 105 - DNA, 18 bp, synthetic construct
  misc_feature 1..18: note = NCgl1874_F
  source 1..18: mol_type = other DNA
ccatgaggcgctcgtagc

SEQ ID NO: 106 - DNA, 18 bp, synthetic construct
  misc_feature 1..18: note = NCgl1874_R
  source 1..18: mol_type = other DNA
agtctccgatcctgtccg

SEQ ID NO: 107 - DNA, 18 bp, synthetic construct
  misc_feature 1..18: note = NCgl2245_F
  source 1..18: mol_type = other DNA
ttggctgcctcaataatc

SEQ ID NO: 108 - DNA, 18 bp, synthetic construct
  misc_feature 1..18: note = NCgl2245_R
  source 1..18: mol_type = other DNA
aatatcttcctcacgatc

SEQ ID NO: 109 - DNA, 18 bp, synthetic construct
  misc_feature 1..18: note = NCgl2580_F
  source 1..18: mol_type = other DNA
cccgtcgcgcgagtcgag

SEQ ID NO: 110 - DNA, 18 bp, synthetic construct
  misc_feature 1..18: note = NCgl2580_R
  source 1..18: mol_type = other DNA
cagcagtgcgtcgcctgc

SEQ ID NO: 111 - DNA, 18 bp, synthetic construct
  misc_feature 1..18: note = NCgl2629_F
  source 1..18: mol_type = other DNA
ttggctgctctttagagg

SEQ ID NO: 112 - DNA, 18 bp, synthetic construct
  misc_feature 1..18: note = NCgl2629_R
  source 1..18: mol_type = other DNA
ctgccgacagaaggcacg

SEQ ID NO: 113 - DNA, 18 bp, synthetic construct
  misc_feature 1..18: note = NCgl2863_F
  source 1..18: mol_type = other DNA
tagcccacgccacgcacg

SEQ ID NO: 114 - DNA, 20 bp, synthetic construct
  misc_feature 1..20: note = NCgl2863_R
  source 1..20: mol_type = other DNA
gaaatcaaaaaccctgctca

SEQ ID NO: 115 - DNA, 5802 bp, synthetic construct
  misc_feature 1..5802: note = pDC24 vector
  source 1..5802: mol_type = other DNA
gttcgcttgctgtccataaaaccgcccagtctagctatcgccatgtaagcccactgcaagctacctgctttctctttgcgcttgcgttttcccttgtccagatagcccagtagctgacattcatccggggtcagcaccgtttctgcggactggctttctacgtgttccgcttcctttagcagcccttgcgccctgagtgcttgcggcagcgtgaagctagcttttatcgccattcgccattcaggctgcgcaactgttgggaagggcgatcggtgcgggcctcttcgctattacgccagctggcgaaagggggatgtgctgcaaggcgattaagttgggtaacgccagggttttcccagtcacgacgttgtaaaacgacggccagtgaattcgagctcggtacccggggatcctctagagtcgacctgcaggcatgcaagcttggcgtaatcatggtcatagctgtttcctgtgtgaaattgttatccgctcacaattccacacaacatacgagccggaagcataaagtgtaaagcctggggtgcctaatgagtgagctaactcacattaattgcgttgcgctcactgcccgctttccagtcgggaaacctgtcgtgccagctgcattaatgaatcggccaacgcgcggggagaggcggtttgcgtattgggcgctcttccgcttcctcgctcactgactcgctgcgctcggtcgttcggctgcggcgagcggtatcagctcactcaaaggcggtaatacggttatccacagaatcaggggataacgcaggaaagaacatgtgagcaaaaggccagcaaaaggccaggaaccgtaaaaaggccgcgttgctggcgtttttccataggctccgcccccctgacgagcatcacaaaaatcgacgctcaagtcagaggtggcgaaacccgacaggactataaagataccaggcgtttccccctggaagctccctcgtgcgctctcctgttccgaccctgccgcttaccggatacctgtccgcctttctcccttcgggaagcgtggcgctttctcaatgctcacgctgtaggtatctcagttcggtgtaggtcgttcgctccaagctgggctgtgtgcacgaaccccccgttcagcccgaccgctgcgccttatccggtaactatcgtcttgagtccaacccggtaagacacgacttatcgccactggcagcagccactggtaacaggattagcagagcgaggtatgtaggcggtgctacagagttcttgaagtggtggcctaactacggctacactagaaggacagtatttggtatctgcgctctgctgaagccagttaccttcggaaaaagagttggtagctcttgatccggcaaacaaaccaccgctggtagcggtggtttttttgtttgcaagcagcagattacgcgcagaaaaaaaggatctcaagaagatcctttgatcttttctacggggtctgacgctcagtggaacgaaaactcacgttaagggattttggtcatgagattatcaaaaaggatcttcacctagatccttttggggtgggcgaagaactccagcatgagatccccgcgctggaggatcatccagccctgatagaaacagaagccactggagcacctcaaaaacaccatcatacactaaatcagtaagttggcagcatcacccgacgcactttgcgccgaataaatacctgtgacggaagatcacttcgcagaataaataaatcctggtgtccctgttgataccgggaagccctgggccaacttttggcgaaaatgagacgttgatcggcacgtaagaggttccaactttcaccataatgaaataagatcactaccgggcgtattttttgagttatcgagattttcaggagctgatagaaacagaagccactggagcacctcaaaaacaccatcatacactaaatcagtaagttggcagcatcacccgacgcactttgcgccgaataaatacctgtgacggaagatcacttcgcagaataaataaatcctggtgtccctgttgataccgggaagccctgggccaacttttggcgaaaatgagacgttgatcggcacgtaagaggttccaactttcaccataatgaaataagatcactaccgggcgtattttttgagttatcgagattttcaggagctctttggcatcgtctctcgcctgtcccctcagttcagtaatttcctgcatttgcctgtttccagtcggtagatattccacaaaacagcagggaagcagcgcttttccgctgcataaccctgcttcggggtcattatagcgattttttcggtatatccatcctttttcgcacgatatacaggattttgccaaagggttcgtgtagactttccttggtgtatccaacggcgtcagccgggcaggataggtgaagtaggcccacccgcgagcgggtgttccttcttcactgtcccttattcgcacctggcggtgctcaacgggaatcctgctctgcgaggctggccggctaccgccggcgtaacagatgagggcaagcggatggctgatgaaaccaagccaaccaggaagggcagcccacctatcaaggtgtactgccttccagacgaacgaagagcgattgaggaaaaggcggcggcggccggcatgagcctgtcggcctacctgctggccgtcggccagggctacaaaatcacgggcgtcgtggactatgagcacgtccgcgagggcgtcccggaaaacgattccgaagcccaacctttcatagaaggcggcggtggaatcgaaatctcgtgatggcaggttgggcgtcgcttggtcggtcatttcgaaaaaggttaggaatacggttagccatttgcctgcttttatatagttcatatgggattcacctttatgttgataagaaataaaagaaaatgccaataggatatcggcattttcttttgcgtttttatttgttaactgttaattgtccttgttcaaggatgctgtctttgacaacagatgttttcttgcctttgatgttcagcaggaagctcggcgcaaacgttgattgtttgtctgcgtagaatcctctgtttgtcatatagcttgtaatcacgacattgtttcctttcgcttgaggtacagcgaagtgtgagtaagtaaaggttacatcgttaggcggatcaagatccatttttaacacaaggccagttttgttcagcggcttgtatgggccagttaaagaattagaaacataaccaagcatgtaaatatcgttagacgtaatgccgtcaatcgtcatttttgatccgcgggagtcagtgaacaggtaccatttgccgttcattttaaagacgttcgcgcgttcaatttcatctgttactgtgttagatgcaatcagcggtttcatcacttttttcagtgtgtaatcatcgtttagctcaatcataccgagagcgccgtttgctaactcagccgtgcgttttttatcgctttgcagaagtttttgactttcttgacggaagaatgatgtgcttttgccatagtatgctttgttaaataaagattcttcgccttggtagccatcttcagttccagtgtttgcttcaaatactaagtatttgtggcctttatcttctacgtagtgaggatctctcagcgtatggttgtcgcctgagctgtagttgccttcatcgatgaactgctgtacattttgatacgtttttccgtcaccgtcaaagattgatttataatcctctacaccgttgatgttcaaagagctgtctgatgctgatacgttaacttgtgcagttgtcagtgtttgtttgccgtaatgtttaccggagaaatcagtgtagaataaacggatttttccgtcagatgtaaatgtggctgaacctgaccattcttgtgtttggtcttttaggatagaatcatttgcatcgaatttgtcgctgtctttaaagacgcggccagcgtttttccagctgtcaatagaagtttcgccgactttttgatagaacatgtaaatcgatgtgtcatccgcatttttaggatctccggctaatgcaaagacgatgtggtagccgtgatagtttgcgacagtgccgtcagcgttttgtaatggccagctgtcccaaacgtccaggccttttgcagaagagatatttttaattgtggacgaatcaaattcagaaacttgatatttttcatttttttgctgttcagggatttgcagcatatcatggcgtgtaatatgggaaatgccgtatgtttccttatatggcttttggttcgtttctttcgcaaacgcttgagttgcgcctcctgccagcagtgcggtagtaaaggttaatactgttgcttgttttgcaaactttttgatgttcatcgttcatgtctccttttttatgtactgtgttagcggtctgcttcttccagccctcctgtttgaagatggcaagttagttacgcacaataaaaaaagacctaaaatatgtaaggggtgacgccaaagtatacactttgccctttacacattttaggtcttgcctgctttatcagtaacaaacccgcgcgatttacttttcgacctcattctattagactctcgtttggattgcaactggtctattttcctcttttgtttgatagaaaatcataaaaggatttgcagactacgggcctaaagaactaaaaaatctatctgtttcttttcattctctgtattttttatagtttctgttgcatgggcataaagttgcctttttaatcacaattcagaaaatatcataatatctcatttcactaaataatagtgaacggcaggtatatgtgatgggttaaaaaggatcaccccagagtcccgctcagaagaactcgtcaagaaggcgatagaaggcgatgcgctgcgaatcgggagcggcgataccgtaaagcacgaggaagcggtcagcccattcgccgccaagctcttcagcaatatcacgggtagccaacgctatgtcctgatagcggtccgccacacccagccggccacagtcgatgaatccagaaaagcggccattttccaccatgatattcggcaagcaggcatcgccatgggtcacgacgagatcctcgccgtcgggcatccgcgccttgagcctggcgaacagttcggctggcgcgagcccctgatgctcttcgtccagatcatcctgatcgacaagaccggcttccatccgagtacgtgctcgctcgatgcgatgtttcgcttggtggtcgaatgggcaggtagccggatcaagcgtatgcagccgccgcattgcatcagccatgatggatactttctcggcaggagcaaggtgagatgacaggagatcctgccccggcacttcgcccaatagcagccagtcccttcccgcttcagtgacaacgtcgagacagctgcgcaaggaacgcccgtcgtggccagccacgatagccgcgctgcctcgtcttggagttcattcagggcaccggacaggtcggtcttgacaaaaagaaccgggcgcccctgcgctgacagccggaacacggcggcatcagagcagccgattgtctgttgtgcccagtcatagccgaatagcctctccacccaagcggccggagaacctgcgtgcaatccatcttgttcaatcatgcgaaacgatcctcatcctgtctcttgatcagatcttgatcccctgcgccatcagatccttggcggcaagaaagccatccagtttactttgcagggcttcccaaccttaccagagggcgccccagctggcaattccg

SEQ ID NO: 116 - protein, 469 aa, synthetic construct
  REGION 1..469: note = wild type protein of gene NCgl0658
MAKRIVIIGGGPAGYEAALAGAKYGAEVTVIEDVGVGGSAVTMDCVPSKSFIAGTGIKTDLRRADDMGLNRGLGKAHLEIDALNIRVKDLAKAQSEDILGQLQRSDVRMINGVGRFDDYNTKQTTHYIKVTHSDGSEETVECDLVLVATGATPRILKGAEPDGERILTWRQVYDIEELPTHLIVVGSGVTGAEFVSAFAELGVKVTMVASRDRILPHDDADAADVLETVLAERGVSLEKHARVESVTRTEDGGVCVRTADGREIYGSHALMTVGSIPNTADLGLENIGVELAPSGHIKVDRVSRTNIPGVYAAGDCTDLFPLASVAAMQGRIAMYHALGEGVSPIRLKTVATAVFTRPEIAAVGITHAQVDSGEVSARVIVLPLATNPRAKMRSLRHGFVKLFCRRNSGLIIGGVVVAPTASELILPIAVAVTNRLTVADLADTFAVYPSLSGSITEAARQLVQHDDLG

SEQ ID NO: 117 - protein, 483 aa, synthetic construct
  REGION 1..483: note = wild type protein of gene NCgl1165
MTTALEEQNAQQAATAGRVVRVIGAVVDVEFPRGELPALYNALTVEVTLESVKKTVVLEVAQHLGDNLIRTIAMAPTDGLVRGAAVTDTARPISVPVGDVVKGHVFNALGDCLDDVSLNNNPEIERWGIHREPPSFDQLEGKTEILETGIKVIDLLTPYVKGGKIGLFGGAGVGKTVLIQEMITRIAREFSGTSVFAGVGERTREGTDLFLEMEEMGVLQDTALVFGQMDEPPGVRMRVALSGLTMAEYFRDVQNQDVLLFIDNIFRFTQAGSEVSTLLGRMPSAVGYQPTLADEMGVLQERITSTKGRSITSLQAVYVPADDYTDPAPATTFAHLDATTELDRSIASKGIYPAVNPLTSTSRILEPAIVGERHYEVSQRVIGILQKNKELQDIIAILGMDELSEEDKITVARARRIERFLGQNFFVAEKFTGLPGSYVPLTDTVDAFERICNGDFDHYPDQAFNGLGGLDDVEAAYKKLTGK

SEQ ID NO: 118 - protein, 264 aa, synthetic construct
  REGION 1..264: note = wild type protein of gene NCgl1859
MVSQTERQHAIASLLAPTGAVSVGDLAEHFHVTTETVRRDLRIMESLGLLQRVHGGAISPEPMGTSPPRLKPALGKGMPPEPRVLELAETAVSLITPLARSIFLDSGLACTAIATVLGDPPEDARWTVVTSSPGAVIALSATDATSTVVLHGQVHGNCSSIIGSTAVDMISQLRADIAFVEVDAIQSDTSLCTFFPETIPIKQAMIKNAAFTVAVLSPRSPQDQELQLLKHPFSTLADFDALVTDDHTLDFPVLPDHNFQVVTP